European Patent Specification EP 3 241 842 B1, published January 31, 2024. Title: Display of binding agents. Applicant: F-Star Biotechnologische Forschungs- und Entwicklungsges.m.b.H. Application EP. The sequence listing filed with the application follows.

SEQUENCE LISTING (82 sequences)

SEQ ID NO: 1 - protein, 232 aa, human
EPKSCDKTHTCPPCPAPELLGGPSVFLFPPKPKDTLMISRTPEVTCVVVDVSHEDPEVKFNWYVDGVEVHNAKTKPREEQYNSTYRVVSVLTVLHQDWLNGKEYKCKVSNKALPAPIEKTISKAKGQPREPQVYTLPPSRDELTKNQVSLTCLVKGFYPSDIAVEWESNGQPENNYKTTPPVLDSDGSFFLYSKLTVDKSRWQQGNVFSCSVMHEALHNHYTQKSLSLSPGK

SEQ ID NO: 2 - protein, 237 aa, artificial
  human IgG including randomized amino acid modifications
  misc_feature (144)..(146): Xaa can be any naturally occurring amino acid
  misc_feature (198)..(205): Xaa can be any naturally occurring amino acid
  misc_feature (208)..(209): Xaa can be any naturally occurring amino acid
EPKSCDKTHTCPPCPAPELLGGPSVFLFPPKPKDTLMISRTPEVTCVVVDVSHEDPEVKFNWYVDGVEVHNAKTKPREEQYNSTYRVVSVLTVLHQDWLNGKEYKCKVSNKALPAPIEKTISKAKGQPREPQVYTLPPSRDELXXXQVSLTCLVKGFYPSDIAVEWESNGQPENNYKTTPPVLDSDGSFFLYSKLTVXXXXXXXXRWXXGNVFSCSVMHEALHNHYTQKSLSLSPGK

SEQ ID NO: 3 - DNA, 728 bp, artificial
  DNA Sequence for Cloning of modified IgG
  misc_feature (438)..(439): n is a, c, g, or t
  misc_feature (441)..(442): n is a, c, g, or t
  misc_feature (444)..(445): n is a, c, g, or t
  misc_feature (600)..(601): n is a, c, g, or t
  misc_feature (603)..(604): n is a, c, g, or t
  misc_feature (606)..(607): n is a, c, g, or t
  misc_feature (609)..(610): n is a, c, g, or t
  misc_feature (612)..(613): n is a, c, g, or t
  misc_feature (615)..(616): n is a, c, g, or t
  misc_feature (618)..(619): n is a, c, g, or t
  misc_feature (621)..(622): n is a, c, g, or t
  misc_feature (630)..(631): n is a, c, g, or t
  misc_feature (633)..(634): n is a, c, g, or t
ccatggccgagcccaaatcttgtgacaaaactcacacatgcccaccgtgcccagcacctgaactcctggggggaccgtcagtcttcctcttccccccaaaacccaaggacaccctcatgatctcccggacccctgaggtcacatgcgtggtggtggacgtgagccacgaagaccctgaggtcaagttcaactggtacgtggacggcgtggaggtgcataatgccaagacaaagccgcgggaggagcagtacaacagcacgtaccgtgtggtcagcgtcctcaccgtcctgcaccaggactggctgaatggcaaggagtacaagtgcaaggtctccaacaaagccctcccagcccccatcgagaaaaccatctccaaagccaaagggcagcctcgagaaccacaggtgtacaccctgcccccatcccgtgacgagctcnnsnnsnnscaagtcagcctgacctgcctggtcaaaggcttctatcccagcgacatcgccgtggagtgggagagcaatgggcagccggagaacaactacaagaccacgcctcccgtgctggactccgacggctccttcttcctctacagcaagcttaccgtgnnsnnsnnsnnsnnsnnsnnsnnsaggtggnnsnnsgggaacgtcttctcatgctccgtgatgcatgaggctctgcacaaccactacacacagaagagcctctccctgtctccgggtaaagcggccgca

SEQ ID NO: 4 - DNA, 33 bp, artificial
  PCR primer EPKSNCO
ccatggccgagcccaaatcttgtgacaaaactc

SEQ ID NO: 5 - DNA, 30 bp, artificial
  PCR primer CH3LSAC
agtcgagctcgtcacgggatgggggcaggg

SEQ ID NO: 6 - DNA, 41 bp, artificial
  PCR primer CH3CSAC
  misc_feature (11)..(12): n is a, c, g, or t
  misc_feature (14)..(15): n is a, c, g, or t
  misc_feature (17)..(18): n is a, c, g, or t
gtacgagctcnnsnnsnnscaagtcagcctgacctgcctgg

SEQ ID NO: 7 - DNA, 32 bp, artificial
  PCR primer CH3CHIN
tgccaagcttgctgtagaggaagaaggagccg

SEQ ID NO: 8 - DNA, 59 bp, artificial
  PCR primer CH3RHIN
  misc_feature (17)..(18): n is a, c, g, or t
  misc_feature (20)..(21): n is a, c, g, or t
  misc_feature (23)..(24): n is a, c, g, or t
  misc_feature (32)..(33): n is a, c, g, or t
  misc_feature (35)..(36): n is a, c, g, or t
tgccaagcttaccgtgnnsnnsnnsaggtggnnsnnsgggaacgtcttctcatgctccg

SEQ ID NO: 9 - DNA, 33 bp, artificial
  PCR primer CH3RNOT
agttgcggccgctttacccggagacagggagag

SEQ ID NO: 10 - protein, 25 aa, artificial
  junction region
SPGKAAAEQKLISEEDLNGAATVES

SEQ ID NO: 11 - protein, 662 aa, artificial
  amino acid sequence of FcabRGD4L
EPKSCDKTHTCPPCPAPELLGGPSVFLFPPKPKDTLMISRTPEVTCVVVDVSHEDPEVKFNWYVDGVEVHNAKTKPREEQYNSTYRVVSVLTVLHQDWLNGKEYKCKVSNKALPAPIEKTISKAKGQPREPQVYTLPPSRDELTKNQVSLTCLVKGFYPSDIAVEWESNGQPENNYKTTPPVLDSDGSFFLYSKLTVGCRGDCLSRWQQGNVFSCSVMHEALHNHYTQKSLSLSPGKEGGGSAAAEQKLISEEDLNGAATVESCLAKPHTENSFTNVWKDDKTLDRYANYEGCLWNATGVVVCTGDETQCYGTWVPIGLAIPENEGGGSEGGGSEGGGSEGGGTKPPEYGDTPIPGYTYINPLDGTYPPGTEQNPANPNPSLEESQPLNTFMFQNNRFRNRQGALTVYTGTVTQGTDPVKTYYQYTPVSSKAMYDAYWNGKFRDCAFHSGFNEDPFVCEYQGQSSDLPQPPVNAGGGSGGGSGGGSEGGGSEGGGSEGGGSEGGGSGGGSGSGDFDYEKMANANKGAMTENADENALQSDAKGKLDSVATDYGAAIDGFIGDVSGLANGNGATGDFAGSNSQMAQVGDGDNSPLMNNFRQYLPSLPQSVECRPYVFGAGKPYEFSIDCDKINLFRGVFAFLLYVATFMYVFSTFANILHKES

SEQ ID NO: 12 - DNA, 5200 bp, artificial
  vector pHENFcabRGD4
gacgaaagggcctcgtgatacgcctatttttataggttaatgtcatgataataatggtttcttagacgtcaggtggcacttttcggggaaatgtgcgcggaacccctatttgtttatttttctaaatacattcaaatatgtatccgctcatgagacaataaccctgataaatgcttcaataatattgaaaaaggaagagtatgagtattcaacatttccgtgtcgcccttattcccttttttgcggcattttgccttcctgtttttgctcacccagaaacgctggtgaaagtaaaagatgctgaagatcagttgggtgcacgagtgggttacatcgaactggatctcaacagcggtaagatccttgagagttttcgccccgaagaacgttttccaatgatgagcacttttaaagttctgctatgtggcgcggtattatcccgtattgacgccgggcaagagcaactcggtcgccgcatacactattctcagaatgacttggttgagtactcaccagtcacagaaaagcatcttacggatggcatgacagtaagagaattatgcagtgctgccataaccatgagtgataacactgcggccaacttacttctgacaacgatcggaggaccgaaggagctaaccgcttttttgcacaacatgggggatcatgtaactcgccttgatcgttgggaaccggagctgaatgaagccataccaaacgacgagcgtgacaccacgatgcctgtagcaatggcaacaacgttgcgcaaactattaactggcgaactacttactctagcttcccggcaacaattaatagactggatggaggcggataaagttgcaggaccacttctgcgctcggcccttccggctggctggtttattgctgataaatctggagccggtgagcgtgggtctcgcggtatcattgcagcactggggccagatggtaagccctcccgtatcgtagttatctacacgacggggagtcaggcaactatggatgaacgaaatagacagatcgctgagataggtgcctcactgattaagcattggtaactgtcagaccaagtttactcatatatactttagattgatttaaaacttcatttttaatttaaaaggatctaggtgaagatcctttttgataatctcatgaccaaaatcccttaacgtgagttttcgttccactgagcgtcagaccccgtagaaaagatcaaaggatcttcttgagatcctttttttctgcgcgtaatctgctgcttgcaaacaaaaaaaccaccgctaccagcggtggtttgtttgccggatcaagagctaccaactctttttccgaaggtaactggcttcagcagagcgcagataccaaatactgtccttctagtgtagccgtagttaggccaccacttcaagaactctgtagcaccgcctacatacctcgctctgctaatcctgttaccagtggctgctgccagtggcgataagtcgtgtcttaccgggttggactcaagacgatagttaccggataaggcgcagcggtcgggctgaacggggggttcgtgcacacagcccagcttggagcgaacgacctacaccgaactgagatacctacagcgtgagcattgagaaagcgccacgcttcccgaagggagaaaggcggacaggtatccggtaagcggcagggtcggaacaggagagcgcacgagggagcttccagggggaaacgcctggtatctttatagtcctgtcgggtttcgccacctctgacttgagcgtcgatttttgtgatgctcgtcaggggggcggagcctatggaaaaacgccagcaacgcggcctttttacggttcctggccttttgctggccttttgctcacatgttctttcctgcgttatcccctgattctgtggataaccgtattaccgcctttgagtgagctgataccgctcgccgcagccgaacgaccgagcgcagcgagtcagtgagcgaggaagcggaagagcgcccaatacgcaaaccgcctctccccgcgcgttggccgattcattaatgcagctggcacgacaggtttcccgactggaaagcgggcagtgagcgcaacgcaattaatgtgagttagctcactcattaggcaccccaggctttacactttatgcttccggctcgtatgttgtgtggaattgtgagcggataacaatttcacacaggaaacagctatgaccatgattacgccaagcttaagcttgcatgcaaattctatttcaaggagacagtcataatgaaatacctattgcctacggcagccgctggattgttattactcgcggcccagccggccatggccgagcccaaatcttgtgacaaaactcacacatgcccaccgtgcccagcacctgaactcctggggggaccgtcagtcttcctcttccccccaaaacccaaggacaccctcatgatctcccggacccctgaggtcacatgcgtggtggtggacgtgagccacgaagaccctgaggtcaagttcaactggtacgtggacggcgtggaggtgcataatgccaagacaaagccgcgggaggagcagtacaacagcacgtaccgtgtggtcagcgtcctcaccgtcctgcaccaggactggctgaatggcaaggagtacaagtgcaaggtctccaacaaagccctcccagcccccatcgagaaaaccatctccaaagccaaagggcagccccgagaaccacaggtgtacaccctgcccccatcccgggatgagctgaccaagaaccaggtcagcctgacctgcctggtcaaaggcttctatcccagcgacatcgccgtggagtgggagagcaatgggcagccggagaacaactacaagaccacgcctcccgtgctggactccgacggctccttcttcctctacagcaagcttaccgtgggttgccgcggtgattgtctgagcaggtggcagcaggggaacgtcttctcatgctccgtgatgcatgaggctctgcacaaccactacacgcagaagagcctctccctgtctccgggtaaagcggccgcagaacaaaaactcatctcagaagaggatctgaatggggccgcatagactgttgaaagttgtttagcaaaacctcatacagaaaattcatttactaacgtctggaaagacgacaaaactttagatcgttacgctaactatgagggctgtctgtggaatgctacaggcgttgtggtttgtactggtgacgaaactcagtgttacggtacatgggttcctattgggcttgctatccctgaaaatgagggtggtggctctgagggtggcggttctgagggtggcggttctgagggtggcggtactaaacctcctgagtacggtgatacacctattccgggctatacttatatcaaccctctcgacggcacttatccgcctggtactgagcaaaaccccgctaatcctaatccttctcttgaggagtctcagcctcttaatactttcatgtttcagaataataggttccgaaataggcagggtgcattaactgtttatacgggcactgttactcaaggcactgaccccgttaaaacttattaccagtacactcctgtatcatcaaaagccatgtatgacgcttactggaacggtaaattcagagactgcgctttccattctggctttaatgaggatccattcgtttgtgaatatcaaggccaatcgtctgacctgcctcaacctcctgtcaatgctggcggcggctctggtggtggttctggtggcggctctgagggtggcggctctgagggtggcggttctgagggtggcggctctgagggtggcggttccggtggcggctccggttccggtgattttgattatgaaaaaatggcaaacgctaataagggggctatgaccgaaaatgccgatgaaaacgcgctacagtctgacgctaaaggcaaacttgattctgtcgctactgattacggtgctgctatcgatggtttcattggtgacgtttccggccttgctaatggtaatggtgctactggtgattttgctggctctaattcccaaatggctcaagtcggtgacggtgataattcacctttaatgaataatttccgtcaatatttaccttctttgcctcagtcggttgaatgtcgcccttatgtctttggcgctggtaaaccatatgaattttctattgattgtgacaaaataaacttattccgtggtgtctttgcgtttcttttatatgttgccacctttatgtatgtattttcgacgtttgctaacatactgcataaggagtcttaataagaattcactggccgtcgttttacaacgtcgtgactgggaaaaccctggcgttacccaacttaatcgccttgcagcacatccccctttcgccagctggcgtaatagcgaagaggcccgcaccgatcgcccttcccaacagttgcgcagcctgaatggcgaatggcgcctgatgcggtattttctccttacgcatctgtgcggtatttcacaccgcacgtcaaagcaaccatagtacgcgccctgtagcggcgcattaagcgcggcgggtgtggtggttacgcgcagcgtgaccgctacacttgccagcgccctagcgcccgctcctttcgctttcttcccttcctttctcgccacgttcgccggctttccccgtcaagctctaaatcgggggctccctttagggttccgatttagtgctttacggcacctcgaccccaaaaaacttgatttgggtgatggttcacgtagtgggccatcgccctgatagacggtttttcgccctttgacgttggagtccacgttctttaatagtggactcttgttccaaactggaacaacactcaaccctatctcgggctattcttttgatttataagggattttgccgatttcggcctattggttaaaaaatgagctgatttaacaaaaatttaacgcgaattttaacaaaatattaacgtttacaattttatggtgcactctcagtacaatctgctctgatgccgcatagttaagccagccccgacacccgccaacacccgctgacgcgccctgacgggcttgtctgctcccggcatccgcttacagacaagctgtgaccgtctccgggagctgcatgtgtcagaggttttcaccgtcatcaccgaaacgcgcga

SEQ ID NO: 13 - DNA, 48 bp, artificial
  CH3rlink
actagcggccgcagagccaccaccctccttacccggagacagggagag

SEQ ID NO: 14 - DNA, 5215 bp, artificial
  vector pHENFcabRGD4L
gacgaaagggcctcgtgatacgcctatttttataggttaatgtcatgataataatggtttcttagacgtcaggtggcacttttcggggaaatgtgcgcggaacccctatttgtttatttttctaaatacattcaaatatgtatccgctcatgagacaataaccctgataaatgcttcaataatattgaaaaaggaagagtatgagtattcaacatttccgtgtcgcccttattcccttttttgcggcattttgccttcctgtttttgctcacccagaaacgctggtgaaagtaaaagatgctgaagatcagttgggtgcacgagtgggttacatcgaactggatctcaacagcggtaagatccttgagagttttcgccccgaagaacgttttccaatgatgagcacttttaaagttctgctatgtggcgcggtattatcccgtattgacgccgggcaagagcaactcggtcgccgcatacactattctcagaatgacttggttgagtactcaccagtcacagaaaagcatcttacggatggcatgacagtaagagaattatgcagtgctgccataaccatgagtgataacactgcggccaacttacttctgacaacgatcggaggaccgaaggagctaaccgcttttttgcacaacatgggggatcatgtaactcgccttgatcgttgggaaccggagctgaatgaagccataccaaacgacgagcgtgacaccacgatgcctgtagcaatggcaacaacgttgcgcaaactattaactggcgaactacttactctagcttcccggcaacaattaatagactggatggaggcggataaagttgcaggaccacttctgcgctcggcccttccggctggctggtttattgctgataaatctggagccggtgagcgtgggtctcgcggtatcattgcagcactggggccagatggtaagccctcccgtatcgtagttatctacacgacggggagtcaggcaactatggatgaacgaaatagacagatcgctgagataggtgcctcactgattaagcattggtaactgtcagaccaagtttactcatatatactttagattgatttaaaacttcatttttaatttaaaaggatctaggtgaagatcctttttgataatctcatgaccaaaatcccttaacgtgagttttcgttccactgagcgtcagaccccgtagaaaagatcaaaggatcttcttgagatcctttttttctgcgcgtaatctgctgcttgcaaacaaaaaaaccaccgctaccagcggtggtttgtttgccggatcaagagctaccaactctttttccgaaggtaactggcttcagcagagcgcagataccaaatactgtccttctagtgtagccgtagttaggccaccacttcaagaactctgtagcaccgcctacatacctcgctctgctaatcctgttaccagtggctgctgccagtggcgataagtcgtgtcttaccgggttggactcaagacgatagttaccggataaggcgcagcggtcgggctgaacggggggttcgtgcacacagcccagcttggagcgaacgacctacaccgaactgagatacctacagcgtgagcattgagaaagcgccacgcttcccgaagggagaaaggcggacaggtatccggtaagcggcagggtcggaacaggagagcgcacgagggagcttccagggggaaacgcctggtatctttatagtcctgtcgggtttcgccacctctgacttgagcgtcgatttttgtgatgctcgtcaggggggcggagcctatggaaaaacgccagcaacgcggcctttttacggttcctggccttttgctggccttttgctcacatgttctttcctgcgttatcccctgattctgtggataaccgtattaccgcctttgagtgagctgataccgctcgccgcagccgaacgaccgagcgcagcgagtcagtgagcgaggaagcggaagagcgcccaatacgcaaaccgcctctccccgcgcgttggccgattcattaatgcagctggcacgacaggtttcccgactggaaagcgggcagtgagcgcaacgcaattaatgtgagttagctcactcattaggcaccccaggctttacactttatgcttccggctcgtatgttgtgtggaattgtgagcggataacaatttcacacaggaaacagctatgaccatgattacgccaagcttaagcttgcatgcaaattctatttcaaggagacagtcataatgaaatacctattgcctacggcagccgctggattgttattactcgcggcccagccggccatggccgagcccaaatcttgtgacaaaactcacacatgcccaccgtgcccagcacctgaactcctggggggaccgtcagtcttcctcttccccccaaaacccaaggacaccctcatgatctcccggacccctgaggtcacatgcgtggtggtggacgtgagccacgaagaccctgaggtcaagttcaactggtacgtggacggcgtggaggtgcataatgccaagacaaagccgcgggaggagcagtacaacagcacgtaccgtgtggtcagcgtcctcaccgtcctgcaccaggactggctgaatggcaaggagtacaagtgcaaggtctccaacaaagccctcccagcccccatcgagaaaaccatctccaaagccaaagggcagccccgagaaccacaggtgtacaccctgcccccatcccgggatgagctgaccaagaaccaggtcagcctgacctgcctggtcaaaggcttctatcccagcgacatcgccgtggagtgggagagcaatgggcagccggagaacaactacaagaccacgcctcccgtgctggactccgacggctccttcttcctctacagcaagcttaccgtgggttgccgcggtgattgtctgagcaggtggcagcaggggaacgtcttctcatgctccgtgatgcatgaggctctgcacaaccactacacgcagaagagcctctccctgtctccgggtaaggagggtggtggctctgcggccgcagaacaaaaactcatctcagaagaggatctgaatggggccgcatagactgttgaaagttgtttagcaaaacctcatacagaaaattcatttactaacgtctggaaagacgacaaaactttagatcgttacgctaactatgagggctgtctgtggaatgctacaggcgttgtggtttgtactggtgacgaaactcagtgttacggtacatgggttcctattgggcttgctatccctgaaaatgagggtggtggctctgagggtggcggttctgagggtggcggttctgagggtggcggtactaaacctcctgagtacggtgatacacctattccgggctatacttatatcaaccctctcgacggcacttatccgcctggtactgagcaaaaccccgctaatcctaatccttctcttgaggagtctcagcctcttaatactttcatgtttcagaataataggttccgaaataggcagggtgcattaactgtttatacgggcactgttactcaaggcactgaccccgttaaaacttattaccagtacactcctgtatcatcaaaagccatgtatgacgcttactggaacggtaaattcagagactgcgctttccattctggctttaatgaggatccattcgtttgtgaatatcaaggccaatcgtctgacctgcctcaacctcctgtcaatgctggcggcggctctggtggtggttctggtggcggctctgagggtggcggctctgagggtggcggttctgagggtggcggctctgagggtggcggttccggtggcggctccggttccggtgattttgattatgaaaaaatggcaaacgctaataagggggctatgaccgaaaatgccgatgaaaacgcgctacagtctgacgctaaaggcaaacttgattctgtcgctactgattacggtgctgctatcgatggtttcattggtgacgtttccggccttgctaatggtaatggtgctactggtgattttgctggctctaattcccaaatggctcaagtcggtgacggtgataattcacctttaatgaataatttccgtcaatatttaccttctttgcctcagtcggttgaatgtcgcccttatgtctttggcgctggtaaaccatatgaattttctattgattgtgacaaaataaacttattccgtggtgtctttgcgtttcttttatatgttgccacctttatgtatgtattttcgacgtttgctaacatactgcataaggagtcttaataagaattcactggccgtcgttttacaacgtcgtgactgggaaaaccctggcgttacccaacttaatcgccttgcagcacatccccctttcgccagctggcgtaatagcgaagaggcccgcaccgatcgcccttcccaacagttgcgcagcctgaatggcgaatggcgcctgatgcggtattttctccttacgcatctgtgcggtatttcacaccgcacgtcaaagcaaccatagtacgcgccctgtagcggcgcattaagcgcggcgggtgtggtggttacgcgcagcgtgaccgctacacttgccagcgccctagcgcccgctcctttcgctttcttcccttcctttctcgccacgttcgccggctttccccgtcaagctctaaatcgggggctccctttagggttccgatttagtgctttacggcacctcgaccccaaaaaacttgatttgggtgatggttcacgtagtgggccatcgccctgatagacggtttttcgccctttgacgttggagtccacgttctttaatagtggactcttgttccaaactggaacaacactcaaccctatctcgggctattcttttgatttataagggattttgccgatttcggcctattggttaaaaaatgagctgatttaacaaaaatttaacgcgaattttaacaaaatattaacgtttacaattttatggtgcactctcagtacaatctgctctgatgccgcatagttaagccagccccgacacccgccaacacccgctgacgcgccctgacgggcttgtctgctcccggcatccgcttacagacaagctgtgaccgtctccgggagctgcatgtgtcagaggttttcaccgtcatcaccgaaacgcgcga

SEQ ID NO: 15 - DNA, 5013 bp, artificial
  vector pYD1dX
acggattagaagccgccgagcgggtgacagccctccgaaggaagactctcctccgtgcgtcctcgtcttcaccggtcgcgttcctgaaacgcagatgtgcctcgcgccgcactgctccgaacaataaagattctacaatactagcttttatggttatgaagaggaaaaattggcagtaacctggccccacaaaccttcaaatgaacgaatcaaattaacaaccataggatgataatgcgattagttttttagccttatttctggggtaattaatcagcgaagcgatgatttttgatctattaacagatatataaatgcaaaaactgcataaccactttaactaatactttcaacattttcggtttgtattacttcttattcaaatgtaataaaagtatcaacaaaaaattgttaatatacctctatactttaacgtcaaggagaaaaaaccccggatcggactactagcagctgtaatacgactcactatagggaatattaagctaattctacttcatacattttcaattaagatgcagttacttcgctgtttttcaatattttctgttattgcttcagttttagcacaggaactgacaactatatgcgagcaaatcccctcaccaactttagaatcgacgccgtactctttgtcaacgactactattttggccaacgggaaggcaatgcaaggagtttttgaatattacaaatcagtaacgtttgtcagtaattgcggttctcacccctcaacaactagcaaaggcagccccataaacacacagtatgtttttaagcttctgcaggctagtggtggtggtggttctggtggtggtggttctggtggtggtggttctgctagcatgactggtggacagcaaatgggtcgggatctgtacgacgatgacgataaggtaccaggatccagtgtggtggaattctgcagatatccagcacagtggcggccgctcgatcgagtctagagggcccttcgaaggtaagcctatccctaaccctctcctcggtctcgattctacgcgtaccggtcatcatcaccatcaccattgagtttaaacccgctgatctgataacaacagtgtagatgtaacaaaatcgactttgttcccactgtacttttagctcgtacaaaatacaatatacttttcatttctccgtaaacaacatgttttcccatgtaatatccttttctatttttcgttccgttaccaactttacacatactttatatagctattcacttctatacactaaaaaactaagacaattttaattttgctgcctgccatatttcaatttgttataaattcctataatttatcctattagtagctaaaaaaagatgaatgtgaatcgaatcctaagagaattgggcaagtgcacaaacaatacttaaataaatactactcagtaataacctatttcttagcatttttgacgaaatttgctattttgttagagtcttttacaccatttgtctccacacctccgcttacatcaacaccaataacgccatttaatctaagcgcatcaccaacattttctggcgtcagtccaccagctaacataaaatgtaagctctcggggctctcttgccttccaacccagtcagaaatcgagttccaatccaaaagttcacctgtcccacctgcttctgaatcaaacaagggaataaacgaatgaggtttctgtgaagctgcactgagtagtatgttgcagtcttttggaaatacgagtcttttaataactggcaaaccgaggaactcttggtattcttgccacgactcatctccgtgcagttggacgatatcaatgccgtaatcattgaccagagccaaaacatcctccttaggttgattacgaaacacgccaaccaagtatttcggagtgcctgaactatttttatatgcttttacaagacttgaaattttccttgcaataaccgggtcaattgttctctttctattgggcacacatataatacccagcaagtcagcatcggaatctagagcacattctgcggcctctgtgctctgcaagccgcaaactttcaccaatggaccagaactacctgtgaaattaataacagacatactccaagctgcctttgtgtgcttaatcacgtatactcacgtgctcaatagtcaccaatgccctccctcttggccctctccttttcttttttcgaccgaatttcttgaagacgaaagggcctcgtgatacgcctatttttataggttaatgtcatgataataatggtttcttaggacggatcgcttgcctgtaacttacacgcgcctcgtatcttttaatgatggaataatttgggaatttactctgtgtttatttatttttatgttttgtatttggattttagaaagtaaataaagaaggtagaagagttacggaatgaagaaaaaaaaataaacaaaggtttaaaaaatttcaacaaaaagcgtactttacatatatatttattagacaagaaaagcagattaaatagatatacattcgattaacgataagtaaaatgtaaaatcacaggattttcgtgtgtggtcttctacacagacaagatgaaacaattcggcattaatacctgagagcaggaagagcaagataaaaggtagtatttgttggcgatccccctagagtcttttacatcttcggaaaacaaaaactattttttctttaatttctttttttactttctatttttaatttatatatttatattaaaaaatttaaattataattatttttatagcacgtgatgaaaaggacccaggtggcacttttcggggaaatgtgcgcggaacccctatttgtttatttttctaaatacattcaaatatgtatccgctcatgagacaataaccctgataaatgcttcaataatattgaaaaaggaagagtatgagtattcaacatttccgtgtcgcccttattcccttttttgcggcattttgccttcctgtttttgctcacccagaaacgctggtgaaagtaaaagatgctgaagatcagttgggtgcacgagtgggttacatcgaactggatctcaacagcggtaagatccttgagagttttcgccccgaagaacgttttccaatgatgagcacttttaaagttctgctatgtggcgcggtattatcccgtgttgacgccgggcaagagcaactcggtcgccgcatacactattctcagaatgacttggttgagtactcaccagtcacagaaaagcatcttacggatggcatgacagtaagagaattatgcagtgctgccataaccatgagtgataacactgcggccaacttacttctgacaacgatcggaggaccgaaggagctaaccgcttttttgcacaacatgggggatcatgtaactcgccttgatcgttgggaaccggagctgaatgaagccataccaaacgacgagcgtgacaccacgatgcctgtagcaatggcaacaacgttgcgcaaactattaactggcgaactacttactctagcttcccggcaacaattaatagactggatggaggcggataaagttgcaggaccacttctgcgctcggcccttccggctggctggtttattgctgataaatctggagccggtgagcgtgggtctcgcggtatcattgcagcactggggccagatggtaagccctcccgtatcgtagttatctacacgacgggcagtcaggcaactatggatgaacgaaatagacagatcgctgagataggtgcctcactgattaagcattggtaactgtcagaccaagtttactcatatatactttagattgatttaaaacttcatttttaatttaaaaggatctaggtgaagatcctttttgataatctcatgaccaaaatcccttaacgtgagttttcgttccactgagcgtcagaccccgtagaaaagatcaaaggatcttcttgagatcctttttttctgcgcgtaatctgctgcttgcaaacaaaaaaaccaccgctaccagcggtggtttgtttgccggatcaagagctaccaactctttttccgaaggtaactggcttcagcagagcgcagataccaaatactgtccttctagtgtagccgtagttaggccaccacttcaagaactctgtagcaccgcctacatacctcgctctgctaatcctgttaccagtggctgctgccagtggcgataagtcgtgtcttaccgggttggactcaagacgatagttaccggataaggcgcagcggtcgggctgaacggggggttcgtgcacacagcccagcttggagcgaacgacctacaccgaactgagatacctacagcgtgagcattgagaaagcgccacgcttcccgaagggagaaaggcggacaggtatccggtaagcggcagggtcggaacaggagagcgcacgagggagcttccaggggggaacgcctggtatctttatagtcctgtcgggtttcgccacctctgacttgagcgtcgatttttgtgatgctcgtcaggggggccgagcctatggaaaaacgccagcaacgcggcctttttacggttcctggccttttgctggccttttgctcacatgttctttcctgcgttatcccctgattctgtggataaccgtattaccgcctttgagtgagctgataccgctcgccgcagccgaacgaccgagcgcagcgagtcagtgagcgaggaagcggaagagcgcccaatacgcaaaccgcctctccccgcgcgttggccgattcattaatgcagctggcacgacaggtttcccgactggaaagcgggcagtgagcgcaacgcaattaatgtgagttacctcactcattaggcaccccaggctttacactttatgcttccggctcctatgttgtgtggaattgtgagcggataacaatttcacacaggaaacagctatgaccatgattacgccaagctcggaattaaccctcactaaagggaacaaaagctggctagt

SEQ ID NO: 16 - DNA, 5971 bp, artificial
  vector pYD1dXFc
acggattagaagccgccgagcgggtgacagccctccgaaggaagactctcctccgtgcgtcctcgtcttcaccggtcgcgttcctgaaacgcagatgtgcctcgcgccgcactgctccgaacaataaagattctacaatactagcttttatggttatgaagaggaaaaattggcagtaacctggccccacaaaccttcaaatgaacgaatcaaattaacaaccataggatgataatgcgattagttttttagccttatttctggggtaattaatcagcgaagcgatgatttttgatctattaacagatatataaatgcaaaaactgcataaccactttaactaatactttcaacattttcggtttgtattacttcttattcaaatgtaataaaagtatcaacaaaaaattgttaatatacctctatactttaacgtcaaggagaaaaaaccccggatcggactactagcagctgtaatacgactcactatagggaatattaagctaattctacttcatacattttcaattaagatgcagttacttcgctgtttttcaatattttctgttattgcttcagttttagcacaggaactgacaactatatgcgagcaaatcccctcaccaactttagaatcgacgccgtactctttgtcaacgactactattttggccaacgggaaggcaatgcaaggagtttttgaatattacaaatcagtaacgtttgtcagtaattgcggttctcacccctcaacaactagcaaaggcagccccataaacacacagtatgtttttaagcttctgcaggctagtggtggtggtggttctggtggtggtggttctggtggtggtggttctgctagcatgactggtggacagcaaatgggtcgggatctgtacgacgatgacgataaggtaccaggatccgctagcaccaagggccccagcgtgttccctctggcccccagctccaagagcacctccggcggcaccgccgccctgggctgcctggtgaaggattacttcccagagcccgtgaccgtgagctggaacagcggcgccctgaccagcggcgtgcacacctttcccgccgtgctgcagtccagcggcctgtactccctgagcagcgtggtgaccgtgcccagcagcagcctgggcacccagacctacatctgcaatgtgaaccacaagcccagcaataccaaggtggataagaaggtggagcccaagagcagcgacaagacacacacgtgtcccccatgtcccgcccctgagctgctgggcggcccttccgtgttcctgttccctcccaagccaaaggacaccctgatgatctcccggacccctgaggtgacctgtgtggtggtggacgtgagccacgaggacccagaggtgaagttcaactggtacgtggacggcgtggaggtgcacaacgccaagaccaagcctagagaggagcagtacaacagcacctaccgcgtggtgagcgtgctgaccgtgctgcaccaggattggctgaatggcaaggagtacaagtgcaaggtgagcaacaaggccctgcctgcccccatcgagaagaccatctccaaggccaagggccagcctcgagaaccacaggtgtacaccctgcccccatcccgggatgagctgaccaagaaccaggtcagcctgacctgcctggtcaaaggcttctatcccagcgacatcgccgtggagtgggagagcaatgggcagccggagaacaactacaagaccacgcctcccgtgctggactccgacggctccttcttcctctacagcaagctcaccgtggacaagagcaggtggcagcaggggaacgtcttctcatgctccgtgatgcatgaggctctgcacaaccactacacacagaagagcctctccctgtctccgggtaaatgagcggccgctcgatcgagtctagagggcccttcgaaggtaagcctatccctaaccctctcctcggtctcgattctacgcgtaccggtcatcatcaccatcaccattgagtttaaacccgctgatctgataacaacagtgtagatgtaacaaaatcgactttgttcccactgtacttttagctcgtacaaaatacaatatacttttcatttctccgtaaacaacatgttttcccatgtaatatccttttctatttttcgttccgttaccaactttacacatactttatatagctattcacttctatacactaaaaaactaagacaattttaattttgctgcctgccatatttcaatttgttataaattcctataatttatcctattagtagctaaaaaaagatgaatgtgaatcgaatcctaagagaattgggcaagtgcacaaacaatacttaaataaatactactcagtaataacctatttcttagcatttttgacgaaatttgctattttgttagagtcttttacaccatttgtctccacacctccgcttacatcaacaccaataacgccatttaatctaagcgcatcaccaacattttctggcgtcagtccaccagctaacataaaatgtaagctctcggggctctcttgccttccaacccagtcagaaatcgagttccaatccaaaagttcacctgtcccacctgcttctgaatcaaacaagggaataaacgaatgaggtttctgtgaagctgcactgagtagtatgttgcagtcttttggaaatacgagtcttttaataactggcaaaccgaggaactcttggtattcttgccacgactcatctccgtgcagttggacgatatcaatgccgtaatcattgaccagagccaaaacatcctccttaggttgattacgaaacacgccaaccaagtatttcggagtgcctgaactatttttatatgcttttacaagacttgaaattttccttgcaataaccgggtcaattgttctctttctattgggcacacatataatacccagcaagtcagcatcggaatctagagcacattctgcggcctctgtgctctgcaagccgcaaactttcaccaatggaccagaactacctgtgaaattaataacagacatactccaagctgcctttgtgtgcttaatcacgtatactcacgtgctcaatagtcaccaatgccctccctcttggccctctccttttcttttttcgaccgaatttcttgaagacgaaagggcctcgtgatacgcctatttttataggttaatgtcatgataataatggtttcttaggacggatcgcttgcctgtaacttacacgcgcctcgtatcttttaatgatggaataatttgggaatttactctgtgtttatttatttttatgttttgtatttggattttagaaagtaaataaagaaggtagaagagttacggaatgaagaaaaaaaaataaacaaaggtttaaaaaatttcaacaaaaagcgtactttacatatatatttattagacaagaaaagcagattaaatagatatacattcgattaacgataagtaaaatgtaaaatcacaggattttcgtgtgtggtcttctacacagacaagatgaaacaattcggcattaatacctgagagcaggaagagcaagataaaaggtagtatttgttggcgatccccctagagtcttttacatcttcggaaaacaaaaactattttttctttaatttctttttttactttctatttttaatttatatatttatattaaaaaatttaaattataattatttttatagcacgtgatgaaaaggacccaggtggcacttttcggggaaatgtgcgcggaacccctatttgtttatttttctaaatacattcaaatatgtatccgctcatgagacaataaccctgataaatgcttcaataatattgaaaaaggaagagtatgagtattcaacatttccgtgtcgcccttattcccttttttgcggcattttgccttcctgtttttgctcacccagaaacgctggtgaaagtaaaagatgctgaagatcagttgggtgcacgagtgggttacatcgaactggatctcaacagcggtaagatccttgagagttttcgccccgaagaacgttttccaatgatgagcacttttaaagttctgctatgtggcgcggtattatcccgtgttgacgccgggcaagagcaactcggtcgccgcatacactattctcagaatgacttggttgagtactcaccagtcacagaaaagcatcttacggatggcatgacagtaagagaattatgcagtgctgccataaccatgagtgataacactgcggccaacttacttctgacaacgatcggaggaccgaaggagctaaccgcttttttgcacaacatgggggatcatgtaactcgccttgatcgttgggaaccggagctgaatgaagccataccaaacgacgagcgtgacaccacgatgcctgtagcaatggcaacaacgttgcgcaaactattaactggcgaactacttactctagcttcccggcaacaattaatagactggatggaggcggataaagttgcaggaccacttctgcgctcggcccttccggctggctggtttattgctgataaatctggagccggtgagcgtgggtctcgcggtatcattgcagcactggggccagatggtaagccctcccgtatcgtagttatctacacgacgggcagtcaggcaactatggatgaacgaaatagacagatcgctgagataggtgcctcactgattaagcattggtaactgtcagaccaagtttactcatatatactttagattgatttaaaacttcatttttaatttaaaaggatctaggtgaagatcctttttgataatctcatgaccaaaatcccttaacgtgagttttcgttccactgagcgtcagaccccgtagaaaagatcaaaggatcttcttgagatcctttttttctgcgcgtaatctgctgcttgcaaacaaaaaaaccaccgctaccagcggtggtttgtttgccggatcaagagctaccaactctttttccgaaggtaactggcttcagcagagcgcagataccaaatactgtccttctagtgtagccgtagttaggccaccacttcaagaactctgtagcaccgcctacatacctcgctctgctaatcctgttaccagtggctgctgccagtggcgataagtcgtgtcttaccgggttggactcaagacgatagttaccggataaggcgcagcggtcgggctgaacggggggttcgtgcacacagcccagcttggagcgaacgacctacaccgaactgagatacctacagcgtgagcattgagaaagcgccacgcttcccgaagggagaaaggcggacaggtatccggtaagcggcagggtcggaacaggagagcgcacgagggagcttccaggggggaacgcctggtatctttatagtcctgtcgggtttcgccacctctgacttgagcgtcgatttttgtgatgctcgtcaggggggccgagcctatggaaaaacgccagcaacgcggcctttttacggttcctggccttttgctggccttttgctcacatgttctttcctgcgttatcccctgattctgtggataaccgtattaccgcctttgagtgagctgataccgctcgccgcagccgaacgaccgagcgcagcgagtcagtgagcgaggaagcggaagagcgcccaatacgcaaaccgcctctccccgcgcgttggccgattcattaatgcagctggcacgacaggtttcccgactggaaagcgggcagtgagcgcaacgcaattaatgtgagttacctcactcattaggcaccccaggctttacactttatgcttccggctcctatgttgtgtggaattgtgagcggataacaatttcacacaggaaacagctatgaccatgattacgccaagctcggaattaaccctcactaaagggaacaaaagctggctagt

SEQ ID NO: 17 - DNA, 5657 bp, artificial
  pYD1CH12
acggattagaagccgccgagcgggtgacagccctccgaaggaagactctcctccgtgcgtcctcgtcttcaccggtcgcgttcctgaaacgcagatgtgcctcgcgccgcactgctccgaacaataaagattctacaatactagcttttatggttatgaagaggaaaaattggcagtaacctggccccacaaaccttcaaatgaacgaatcaaattaacaaccataggatgataatgcgattagttttttagccttatttctggggtaattaatcagcgaagcgatgatttttgatctattaacagatatataaatgcaaaaactgcataaccactttaactaatactttcaacattttcggtttgtattacttcttattcaaatgtaataaaagtatcaacaaaaaattgttaatatacctctatactttaacgtcaaggagaaaaaaccccggatcggactactagcagctgtaatacgactcactatagggaatattaagctaattctacttcatacattttcaattaagatgcagttacttcgctgtttttcaatattttctgttattgcttcagttttagcacaggaactgacaactatatgcgagcaaatcccctcaccaactttagaatcgacgccgtactctttgtcaacgactactattttggccaacgggaaggcaatgcaaggagtttttgaatattacaaatcagtaacgtttgtcagtaattgcggttctcacccctcaacaactagcaaaggcagccccataaacacacagtatgtttttaagcttctgcaggctagtggtggtggtggttctggtggtggtggttctggtggtggtggttctgctagcatgactggtggacagcaaatgggtcgggatctgtacgacgatgacgataaggtaccaggatccgctagcaccaagggccccagcgtgttccctctggcccccagctccaagagcacctccggcggcaccgccgccctgggctgcctggtgaaggattacttcccagagcccgtgaccgtgagctggaacagcggcgccctgaccagcggcgtgcacacctttcccgccgtgctgcagtccagcggcctgtactccctgagcagcgtggtgaccgtgcccagcagcagcctgggcacccagacctacatctgcaatgtgaaccacaagcccagcaataccaaggtggataagaaggtggagcccaagagcagcgacaagacacacacgtgtcccccatgtcccgcccctgagctgctgggcggcccttccgtgttcctgttccctcccaagccaaaggacaccctgatgatctcccggacccctgaggtgacctgtgtggtggtggacgtgagccacgaggacccagaggtgaagttcaactggtacgtggacggcgtggaggtgcacaacgccaagaccaagcctagagaggagcagtacaacagcacctaccgcgtggtgagcgtgctgaccgtgctgcaccaggattggctgaatggcaaggagtacaagtgcaaggtgagcaacaaggccctgcctgcccccatcgagaagaccatctccaaggccaagggccagcctcgaggccgctcgatcgagtctagagggcccttcgaaggtaagcctatccctaaccctctcctcggtctcgattctacgcgtaccggtcatcatcaccatcaccattgagtttaaacccgctgatctgataacaacagtgtagatgtaacaaaatcgactttgttcccactgtacttttagctcgtacaaaatacaatatacttttcatttctccgtaaacaacatgttttcccatgtaatatccttttctatttttcgttccgttaccaactttacacatactttatatagctattcacttctatacactaaaaaactaagacaattttaattttgctgcctgccatatttcaatttgttataaattcctataatttatcctattagtagctaaaaaaagatgaatgtgaatcgaatcctaagagaattgggcaagtgcacaaacaatacttaaataaatactactcagtaataacctatttcttagcatttttgacgaaatttgctattttgttagagtcttttacaccatttgtctccacacctccgcttacatcaacaccaataacgccatttaatctaagcgcatcaccaacattttctggcgtcagtccaccagctaacataaaatgtaagctctcggggctctcttgccttccaacccagtcagaaatcgagttccaatccaaaagttcacctgtcccacctgcttctgaatcaaacaagggaataaacgaatgaggtttctgtgaagctgcactgagtagtatgttgcagtcttttggaaatacgagtcttttaataactggcaaaccgaggaactcttggtattcttgccacgactcatctccgtgcagttggacgatatcaatgccgtaatcattgaccagagccaaaacatcctccttaggttgattacgaaacacgccaaccaagtatttcggagtgcctgaactatttttatatgcttttacaagacttgaaattttccttgcaataaccgggtcaattgttctctttctattgggcacacatataatacccagcaagtcagcatcggaatctagagcacattctgcggcctctgtgctctgcaagccgcaaactttcaccaatggaccagaactacctgtgaaattaataacagacatactccaagctgcctttgtgtgcttaatcacgtatactcacgtgctcaatagtcaccaatgccctccctcttggccctctccttttcttttttcgaccgaatttcttgaagacgaaagggcctcgtgatacgcctatttttataggttaatgtcatgataataatggtttcttaggacggatcgcttgcctgtaacttacacgcgcctcgtatcttttaatgatggaataatttgggaatttactctgtgtttatttatttttatgttttgtatttggattttagaaagtaaataaagaaggtagaagagttacggaatgaagaaaaaaaaataaacaaaggtttaaaaaatttcaacaaaaagcgtactttacatatatatttattagacaagaaaagcagattaaatagatatacattcgattaacgataagtaaaatgtaaaatcacaggattttcgtgtgtggtcttctacacagacaagatgaaacaattcggcattaatacctgagagcaggaagagcaagataaaaggtagtatttgttggcgatccccctagagtcttttacatcttcggaaaacaaaaactattttttctttaatttctttttttactttctatttttaatttatatatttatattaaaaaatttaaattataattatttttatagcacgtgatgaaaaggacccaggtggcacttttcggggaaatgtgcgcggaacccctatttgtttatttttctaaatacattcaaatatgtatccgctcatgagacaataaccctgataaatgcttcaataatattgaaaaaggaagagtatgagtattcaacatttccgtgtcgcccttattcccttttttgcggcattttgccttcctgtttttgctcacccagaaacgctggtgaaagtaaaagatgctgaagatcagttgggtgcacgagtgggttacatcgaactggatctcaacagcggtaagatccttgagagttttcgccccgaagaacgttttccaatgatgagcacttttaaagttctgctatgtggcgcggtattatcccgtgttgacgccgggcaagagcaactcggtcgccgcatacactattctcagaatgacttggttgagtactcaccagtcacagaaaagcatcttacggatggcatgacagtaagagaattatgcagtgctgccataaccatgagtgataacactgcggccaacttacttctgacaacgatcggaggaccgaaggagctaaccgcttttttgcacaacatgggggatcatgtaactcgccttgatcgttgggaaccggagctgaatgaagccataccaaacgacgagcgtgacaccacgatgcctgtagcaatggcaacaacgttgcgcaaactattaactggcgaactacttactctagcttcccggcaacaattaatagactggatggaggcggataaagttgcaggaccacttctgcgctcggcccttccggctggctggtttattgctgataaatctggagccggtgagcgtgggtctcgcggtatcattgcagcactggggccagatggtaagccctcccgtatcgtagttatctacacgacgggcagtcaggcaactatggatgaacgaaatagacagatcgctgagataggtgcctcactgattaagcattggtaactgtcagaccaagtttactcatatatactttagattgatttaaaacttcatttttaatttaaaaggatctaggtgaagatcctttttgataatctcatgaccaaaatcccttaacgtgagttttcgttccactgagcgtcagaccccgtagaaaagatcaaaggatcttcttgagatcctttttttctgcgcgtaatctgctgcttgcaaacaaaaaaaccaccgctaccagcggtggtttgtttgccggatcaagagctaccaactctttttccgaaggtaactggcttcagcagagcgcagataccaaatactgtccttctagtgtagccgtagttaggccaccacttcaagaactctgtagcaccgcctacatacctcgctctgctaatcctgttaccagtggctgctgccagtggcgataagtcgtgtcttaccgggttggactcaagacgatagttaccggataaggcgcagcggtcgggctgaacggggggttcgtgcacacagcccagcttggagcgaacgacctacaccgaactgagatacctacagcgtgagcattgagaaagcgccacgcttcccgaagggagaaaggcggacaggtatccggtaagcggcagggtcggaacaggagagcgcacgagggagcttccaggggggaacgcctggtatctttatagtcctgtcgggtttcgccacctctgacttgagcgtcgatttttgtgatgctcgtcaggggggccgagcctatggaaaaacgccagcaacgcggcctttttacggttcctggccttttgctggccttttgctcacatgttctttcctgcgttatcccctgattctgtggataaccgtattaccgcctttgagtgagctgataccgctcgccgcagccgaacgaccgagcgcagcgagtcagtgagcgaggaagcggaagagcgcccaatacgcaaaccgcctctccccgcgcgttggccgattcattaatgcagctggcacgacaggtttcccgactggaaagcgggcagtgagcgcaacgcaattaatgtgagttacctcactcattaggcaccccaggctttacactttatgcttccggctcctatgttgtgtggaattgtgagcggataacaatttcacacaggaaacagctatgaccatgattacgccaagctcggaattaaccctcactaaagggaacaaaagctggctagt

SEQ ID NO: 18 - DNA, 738 bp, artificial
  Fcab01
  misc_feature (449)..(450): n is a, c, g, or t
  misc_feature (452)..(453): n is a, c, g, or t
  misc_feature (455)..(456): n is a, c, g, or t
  misc_feature (611)..(612): n is a, c, g, or t
  misc_feature (614)..(615): n is a, c, g, or t
  misc_feature (617)..(618): n is a, c, g, or t
  misc_feature (620)..(621): n is a, c, g, or t
  misc_feature (623)..(624): n is a, c, g, or t
  misc_feature (626)..(627): n is a, c, g, or t
  misc_feature (629)..(630): n is a, c, g, or t
  misc_feature (632)..(633): n is a, c, g, or t
  misc_feature (641)..(642): n is a, c, g, or t
  misc_feature (644)..(645): n is a, c, g, or t
ggcccagccggccatggccgagcccaaatcttgtgacaaaactcacacatgcccaccgtgcccagcacctgaactcctggggggaccgtcagtcttcctcttccccccaaaacccaaggacaccctcatgatctcccggacccctgaggtcacatgcgtggtggtggacgtgagccacgaagaccctgaggtcaagttcaactggtacgtggacggcgtggaggtgcataatgccaagacaaagccgcgggaggagcagtacaacagcacgtaccgtgtggtcagcgtcctcaccgtcctgcaccaggactggctgaatggcaaggagtacaagtgcaaggtctccaacaaagccctcccagcccccatcgagaaaaccatctccaaagccaaagggcagcctcgagaaccacaggtgtacaccctgcccccatcccgggatgaactgnnbnnbnnbcaggtcagcctgacctgcctggtcaaaggcttctatcccagcgacatcgccgtggagtgggagagcaatgggcagccggagaacaactacaagaccacgcctcccgtgctggactccgacggctccttcttcctctacagcaagctcaccgtgnnbnnbnnbnnbnnbnnbnnbnnbaggtggnnbnnbgggaacgtcttctcatgctccgtgatgcatgaggctctgcacaaccactacacgcagaagagcctctccctgtctccgggtaaagcggccgc

SEQ ID NO: 19 - DNA, 738 bp, artificial
  Fcab02
ggcccagccggccatggccgagcccaaatcttgtgacaaaactcacacatgcccaccgtgcccagcacctgaactcctggggggaccgtcagtcttcctcttccccccaaaacccaaggacaccctcatgatctcccggacccctgaggtcacatgcgtggtggtggacgtgagccacgaagaccctgaggtcaagttcaactggtacgtggacggcgtggaggtgcataatgccaagacaaagccgcgggaggagcagtacaacagcacgtaccgtgtggtcagcgtcctcaccgtcctgcaccaggactggctgaatggcaaggagtacaagtgcaaggtctccaacaaagccctcccagcccccatcgagaaaaccatctccaaagccaaagggcagcctcgagaaccacaggtgtacaccctgcccccatcccgggatgagctgkmtkmtkmtcaggtgagcctgacctgcctggtcaaaggcttctatcccagcgacatcgccgtggagtgggagagcaatgggcagccggagaacaactacaagaccacgcctcccgtgctggactccgacggctccttcttcctctacagcaagctcaccgtgkmtkmtkmtkmtkmtkmtkmtkmtaggtggkmtkmtgggaacgtcttctcatgctccgtgatgcatgaggctctgcacaaccactacacgcagaagagcctctccctgtctccgggtaaagcggccgc

SEQ ID NO: 20 - DNA, 750 bp, artificial
  Fcab03
  misc_feature (449)..(450): n is a, c, g, or t
  misc_feature (452)..(453): n is a, c, g, or t
  misc_feature (455)..(456): n is a, c, g, or t
  misc_feature (617)..(618): n is a, c, g, or t
  misc_feature (620)..(621): n is a, c, g, or t
  misc_feature (623)..(624): n is a, c, g, or t
  misc_feature (626)..(627): n is a, c, g, or t
  misc_feature (629)..(630): n is a, c, g, or t
  misc_feature (632)..(633): n is a, c, g, or t
  misc_feature (635)..(636): n is a, c, g, or t
  misc_feature (638)..(639): n is a, c, g, or t
  misc_feature (653)..(654): n is a, c, g, or t
  misc_feature (656)..(657): n is a, c, g, or t
ggcccagccggccatggccgagcccaaatcttgtgacaaaactcacacatgcccaccgtgcccagcacctgaactcctggggggaccgtcagtcttcctcttccccccaaaacccaaggacaccctcatgatctcccggacccctgaggtcacatgcgtggtggtggacgtgagccacgaagaccctgaggtcaagttcaactggtacgtggacggcgtggaggtgcataatgccaagacaaagccgcgggaggagcagtacaacagcacgtaccgtgtggtcagcgtcctcaccgtcctgcaccaggactggctgaatggcaaggagtacaagtgcaaggtctccaacaaagccctcccagcccccatcgagaaaaccatctccaaagccaaagggcagcctcgagaaccacaggtgtacaccctgcccccttcccgggatgagctgnnbnnbnnbcaggtcagcctgacctgcctggtcaaaggcttctatcccagcgacatcgccgtggagtgggagagcaatgggcagccggagaacaactacaagaccacgcctcccgtgctggactccgacggctccttcttcctctacagcaagctcaccgtgggttctnnbnnbnnbnnbnnbnnbnnbnnbagcggcaggtggnnbnnbgggaacgtcttctcatgctccgtgatgcatgaggctctgcacaaccactacacgcagaagagcctctccctgtctccgggtaaagcggccgc

SEQ ID NO: 21 - DNA, 750 bp, artificial
  Fcab04
ggcccagccggccatggccgagcccaaatcttgtgacaaaactcacacatgcccaccgtgcccagcacctgaactcctggggggaccgtcagtcttcctcttccccccaaaacccaaggacaccctcatgatctcccggacccctgaggtcacatgcgtggtggtggacgtgagccacgaagaccctgaggtcaagttcaactggtacgtggacggcgtggaggtgcataatgccaagacaaagccgcgggaggagcagtacaacagcacgtaccgtgtggtcagcgtcctcaccgtcctgcaccaggactggctgaatggcaaggagtacaagtgcaaggtctccaacaaagccctcccagcccccatcgagaaaaccatctccaaagccaaagggcagcctcgagaaccacaggtgtacaccctgcccccatctcgggatgagctgkmtkmtkmtcaggtcagcctgacctgcctggtcaaaggcttctatcccagcgacatcgccgtggagtgggagagcaatgggcagccggagaacaactacaagaccacgcctcccgtgctggactccgacggctccttcttcctctacagcaagctcaccgtgggttctkmtkmtkmtkmtkmtkmtkmtkmtagcggcaggtggkmtkmtgggaacgtcttctcatgctccgtgatgcatgaggctctgcacaaccactacacgcagaagagcctctccctgtctccgggtaaagcggccgc

SEQ ID NO: 22 - DNA, 738 bp, artificial
  Fcab05
  misc_feature (449)..(450): n is a, c, g, or t
  misc_feature (452)..(453): n is a, c, g, or t
  misc_feature (455)..(456): n is a, c, g, or t
  misc_feature (611)..(612): n is a, c, g, or t
  misc_feature (614)..(615): n is a, c, g, or t
  misc_feature (617)..(618): n is a, c, g, or t
  misc_feature (620)..(621): n is a, c, g, or t
  misc_feature (623)..(624): n is a, c, g, or t
  misc_feature (626)..(627): n is a, c, g, or t
  misc_feature (629)..(630): n is a, c, g, or t
  misc_feature (632)..(633): n is a, c, g, or t
  misc_feature (641)..(642): n is a, c, g, or t
  misc_feature (644)..(645): n is a, c, g, or t
ggcccagccggccatggccgagcccaaatcttgtgacaaaactcacacatgcccaccgtgcccagcacctgaactcctggggggaccgtcagtcttcctcttccccccaaaacccaaggacaccctcatgatctcccggacccctgaggtcacatgcgtggtggtggacgtgagccacgaagaccctgaggtcaagttcaactggtacgtggacggcgtggaggtgcataatgccaagacaaagccgcgggaggagcagtacaacagcacgtaccgtgtggtcagcgtcctcaccgtcctgcaccaggactggctgaatggcaaggagtacaagtgcaaggtctccaacaaagccctcccagcccccatcgagaaaaccatctccaaagccaaagggcagcctcgagaaccacaggtgtacaccctgcccccatcccgtgatgagkmtnnbnnbnnbkmtgtcagcctgacctgcctggtcaaaggcttctatcccagcgacatcgccgtggagtgggagagcaatgggcagccggagaacaactacaagaccacgcctcccgtgctggactccgacggctccttcttcctctacagcaagctcaccgtgnnbnnbnnbnnbnnbnnbnnbnnbaggtggnnbnnbgggaacgtcttctcatgctccgtgatgcatgaggctctgcacaaccactacacgcagaagagcctctccctgtctccgggtaaagcggccgc

SEQ ID NO: 23 - DNA, 738 bp, artificial
  Fcab06
ggcccagccggccatggccgagcccaaatcttgtgacaaaactcacacatgcccaccgtgcccagcacctgaactcctggggggaccgtcagtcttcctcttccccccaaaacccaaggacaccctcatgatctcccggacccctgaggtcacatgcgtggtggtggacgtgagccacgaagaccctgaggtcaagttcaactggtacgtggacggcgtggaggtgcataatgccaagacaaagccgcgggaggagcagtacaacagcacgtaccgtgtggtcagcgtcctcaccgtcctgcaccaggactggctgaatggcaaggagtacaagtgcaaggtctccaacaaagccctcccagcccccatcgagaaaaccatctccaaagccaaagggcagcctcgagaaccacaggtgtacaccctgcccccatcccgggacgagkmtkmtkmtkmtkmtgtcagcctgacctgcctggtcaaaggcttctatcccagcgacatcgccgtggagtgggagagcaatgggcagccggagaacaactacaagaccacgcctcccgtgctggactccgacggctccttcttcctctacagcaagctcaccgtgkmtkmtkmtkmtkmtkmtkmtkmtaggtggkmtkmtgggaacgtcttctcatgctccgtgatgcatgaggctctgcacaaccactacacgcagaagagcctctccctgtctccgggtaaagcggccgc

SEQ ID NO: 24 - DNA, 85 bp, artificial
  PCR primer gapch35
caacaaggccctgcctgcccccatcgagaagaccatctccaaggccaagggccagcctcgagaaccacaggtgtacaccctgccc

SEQ ID NO: 25 - DNA, 99 bp, artificial
  PCR primer gapfcs3
gagaccgaggagagggttagggataggcttaccttcgaagggccctctagactcgatcgagcggccgctcatttacccggagacagggagaggctcttc

SEQ ID NO: 26 - DNA, 79 bp, artificial
  primer Abmut
  misc_feature (43)..(44): n is a, c, g, or t
  misc_feature (46)..(47): n is a, c, g, or t
  misc_feature (49)..(50): n is a, c, g, or t
gaaccacaggtgtacaccctgcccccatcccgggatgagctgnnbnnbnnbcaggtcagcctgacctgcctggtcaaag

SEQ ID NO: 27 - DNA, 79 bp, artificial
  primer Abmut2LR
  misc_feature (40)..(41): n is a, c, g, or t
  misc_feature (43)..(44): n is a, c, g, or t
  misc_feature (46)..(47): n is a, c, g, or t
  misc_feature (49)..(50): n is a, c, g, or t
  misc_feature (52)..(53): n is a, c, g, or t
gaaccacaggtgtacaccctgcccccatcccgggatgagnnbnnbnnbnnbnnbgtcagcctgacctgcctggtcaaag

SEQ ID NO: 28 - DNA, 79 bp, artificial
  primer Abmut1L
  misc_feature (40)..(41): n is a, c, g, or t
  misc_feature (43)..(44): n is a, c, g, or t
  misc_feature (46)..(47): n is a, c, g, or t
  misc_feature (49)..(50): n is a, c, g, or t
gaaccacaggtgtacaccctgcccccatcccgggatgagnnbnnbnnbnnbcaggtcagcctgacctgcctggtcaaag

SEQ ID NO: 29 - DNA, 79 bp, artificial
  primer Abmut1R
  misc_feature (43)..(44): n is a, c, g, or t
  misc_feature (46)..(47): n is a, c, g, or t
  misc_feature (49)..(50): n is a, c, g, or t
  misc_feature (52)..(53): n is a, c, g, or t
gaaccacaggtgtacaccctgcccccatcccgggatgagctgnnbnnbnnbnnbgtcagcctgacctgcctggtcaaag

SEQ ID NO: 30 - protein, 5 aa, artificial
  AB-loop sequence AA143ff
LDNSQ

SEQ ID NO: 31 - protein, 5 aa, artificial
  AB-loop sequence AA143ff
YEGSS

SEQ ID NO: 32 - protein, 5 aa, artificial
  AB-loop sequence AA143ff
YMSAD

SEQ ID NO: 33 - protein, 5 aa, artificial
  AB-loop sequence AA143ff
YRRGD

SEQ ID NO: 34 - protein, 5 aa, artificial
  AB-loop sequence AA143ff
LMSRQ

SEQ ID NO: 35 - protein, 5 aa, artificial
  AB-loop sequence AA143ff
LHLAQ

SEQ ID NO: 36 - protein, 5 aa, artificial
  AB-loop sequence AA143ff
YLSKD

SEQ ID NO: 37 - protein, 5 aa, artificial
  AB-loop sequence AA143ff
YRSGS

SEQ ID NO: 38 - protein, 5 aa, artificial
  AB-loop sequence AA143ff
LRDGQ

SEQ ID NO: 39 - protein, 5 aa, artificial
  AB-loop sequence AA143ff
YSANT

SEQ ID NO: 40 - protein, 5 aa, artificial
  AB-loop sequence AA143ff
YASNT

SEQ ID NO: 41 - protein, 5 aa, artificial
  AB-loop sequence AA143ff
YSDGD

SEQ ID NO: 42 - protein, 5 aa, artificial
  AB-loop sequence AA143ff
YSGGS

SEQ ID NO: 43 - protein, 5 aa, artificial
  AB-loop sequence AA143ff
YGRDS

SEQ ID NO: 44 - protein, 5 aa, artificial
  AB-loop sequence AA143ff
YAGGT

SEQ ID NO: 45 - protein, 5 aa, artificial
  AB-loop sequence AA143ff
YSSDS

SEQ ID NO: 46 - protein, 5 aa, artificial
  AB-loop sequence AA143ff
YHSGS

SEQ ID NO: 47 - protein, 5 aa, artificial
  AB-loop sequence AA143ff
YLTNS

SEQ ID NO: 48 - protein, 5 aa, artificial
  AB-loop sequence AA143ff
YGSEE

SEQ ID NO: 49 - protein, 5 aa, artificial
  AB-loop sequence AA143ff
YRSGE

SEQ ID NO: 50 - protein, 5 aa, artificial
  AB-loop sequence AA143ff
YGTDD

SEQ ID NO: 51 - protein, 12 aa, artificial
  EF-loop sequence AA198ff
IRSSVGSRRWWS

SEQ ID NO: 52 - protein, 12 aa, artificial
  EF-loop sequence AA198ff
ARYSPRMLRWAH

SEQ ID NO: 53 - protein, 12 aa, artificial
  EF-loop sequence AA198ff
SRRDSSLLRWAH

SEQ ID NO: 54 - protein, 12 aa, artificial
  EF-loop sequence AA198ff
APGSKGYRRWAL

SEQ ID NO: 55 - protein, 12 aa, artificial
  EF-loop sequence AA198ff
DKPFWGTSRWSR

SEQ ID NO: 56 - protein, 12 aa, artificial
  EF-loop sequence AA198ff
SINDLINHRWPY

SEQ ID NO: 57 - protein, 12 aa, artificial
  EF-loop sequence AA198ff
MWGSRDYWRWSH

SEQ ID NO: 58 - protein, 12 aa, artificial
  EF-loop sequence AA198ff
NSGSAMMVRWAH

SEQ ID NO: 59 - protein, 12 aa, artificial
  EF-loop sequence AA198ff
QRSRLSRQRWWR

SEQ ID NO: 60 - protein, 12 aa, artificial
  EF-loop sequence AA198ff
ARYSPRMLRWAH

SEQ ID NO: 61 - protein, 12 aa, artificial
  EF-loop sequence AA198ff
ARYSPRMLRWAH

SEQ ID NO: 62 - protein, 12 aa, artificial
  EF-loop sequence AA198ff
ARYSPRMLRWAH

SEQ ID NO: 63 - protein, 12 aa, artificial
  EF-loop sequence AA198ff
ARYSPRMLRWAH

SEQ ID NO: 64 - protein, 12 aa, artificial
  EF-loop sequence AA198ff
ARYSPRMLRWAH

SEQ ID NO: 65 - protein, 12 aa, artificial
  EF-loop sequence AA198ff
ARYSPRMLRWAH

SEQ ID NO: 66 - protein, 12 aa, artificial
  EF-loop sequence AA198ff
ARYSPRMLRWAH

SEQ ID NO: 67 - protein, 12 aa, artificial
  EF-loop sequence AA198ff
ARYSPRMLRWAH

SEQ ID NO: 68 - protein, 12 aa, artificial
  EF-loop sequence AA198ff
ARYSPRMLRWAH

SEQ ID NO: 69 - protein, 12 aa, artificial
  EF-loop sequence AA198ff
ARYSPRMLRWAH

SEQ ID NO: 70 - protein, 12 aa, artificial
  EF-loop sequence AA198ff
ARYSPRMLRWAH

SEQ ID NO: 71 - protein, 12 aa, artificial
  EF-loop sequence AA198ff
ARYSPRMLRWAH

SEQ ID NO: 72 - DNA, 5009 bp, artificial
  vector pYD1
acggattagaagccgccgagcgggtgacagccctccgaaggaagactctcctccgtgcgtcctcgtcttcaccggtcgcgttcctgaaacgcagatgtgcctcgcgccgcactgctccgaacaataaagattctacaatactagcttttatggttatgaagaggaaaaattggcagtaacctggccccacaaaccttcaaatgaacgaatcaaattaacaaccataggatgataatgcgattagttttttagccttatttctggggtaattaatcagcgaagcgatgatttttgatctattaacagatatataaatgcaaaaactgcataaccactttaactaatactttcaacattttcggtttgtattacttcttattcaaatgtaataaaagtatcaacaaaaaattgttaatatacctctatactttaacgtcaaggagaaaaaaccccggatcggactactagcagctgtaatacgactcactatagggaatattaagctaattctacttcatacattttcaattaagatgcagttacttcgctgtttttcaatattttctgttattgcttcagttttagcacaggaactgacaactatatgcgagcaaatcccctcaccaactttagaatcgacgccgtactctttgtcaacgactactattttggccaacgggaaggcaatgcaaggagtttttgaatattacaaatcagtaacgtttgtcagtaattgcggttctcacccctcaacaactagcaaaggcagccccataaacacacagtatgtttttaagcttctgcaggctagtggtggtggtggttctggtggtggtggttctggtggtggtggttctgctagcatgactggtggacagcaaatgggtcgggatctgtacgacgatgacgataaggtaccaggatccagtgtggtggaattctgcagatatccagcacagtggcggccgctcgagtctagagggcccttcgaaggtaagcctatccctaaccctctcctcggtctcgattctacgcgtaccggtcatcatcaccatcaccattgagtttaaacccgctgatctgataacaacagtgtagatgtaacaaaatcgactttgttcccactgtacttttagctcgtacaaaatacaatatacttttcatttctccgtaaacaacatgttttcccatgtaatatccttttctatttttcgttccgttaccaactttacacatactttatatagctattcacttctatacactaaaaaactaagacaattttaattttgctgcctgccatatttcaatttgttataaattcctataatttatcctattagtagctaaaaaaagatgaatgtgaatcgaatcctaagagaattgggcaagtgcacaaacaatacttaaataaatactactcagtaataacctatttcttagcatttttgacgaaatttgctattttgttagagtcttttacaccatttgtctccacacctccgcttacatcaacaccaataacgccatttaatctaagcgcatcaccaacattttctggcgtcagtccaccagctaacataaaatgtaagctctcggggctctcttgccttccaacccagtcagaaatcgagttccaatccaaaagttcacctgtcccacctgcttctgaatcaaacaagggaataaacgaatgaggtttctgtgaagctgcactgagtagtatgttgcagtcttttggaaatacgagtcttttaataactggcaaaccgaggaactcttggtattcttgccacgactcatctccgtgcagttggacgatatcaatgccgtaatcattgaccagagccaaaacatcctccttaggttgattacgaaacacgccaaccaagtatttcggagtgcctgaactatttttatatgcttttacaagacttgaaattttccttgcaataaccgggtcaattgttctctttctattgggcacacatataatacccagcaagtcagcatcggaatctagagcacattctgcggcctctgtgctctgcaagccgcaaactttcaccaatggaccagaactacctgtgaaattaataacagacatactccaagctgcctttgtgtgcttaatcacgtatactcacgtgctcaatagtcaccaatgccctccctcttggccctctccttttcttttttcgaccgaatttcttgaagacgaaagggcctcgtgatacgcctatttttataggttaatgtcatgataataatggtttcttaggacggatcgcttgcctgtaacttacacgcgcctcgtatcttttaatgatggaataatttgggaatttactctgtgtttatttatttttatgttttgtatttggattttagaaagtaaataaagaaggtagaagagttacggaatgaagaaaaaaaaataaacaaaggtttaaaaaatttcaacaaaaagcgtactttacatatatatttattagacaagaaaagcagattaaatagatatacattcgattaacgataagtaaaatgtaaaatcacaggattttcgtgtgtggtcttctacacagacaagatgaaacaattcggcattaatacctgagagcaggaagagcaagataaaaggtagtatttgttggcgatccccctagagtcttttacatcttcggaaaacaaaaactattttttctttaatttctttttttactttctatttttaatttatatatttatattaaaaaatttaaattataattatttttatagcacgtgatgaaaaggacccaggtggcacttttcggggaaatgtgcgcggaacccctatttgtttatttttctaaatacattcaaatatgtatccgctcatgagacaataaccctgataaatgcttcaataatattgaaaaaggaagagtatgagtattcaacatttccgtgtcgcccttattcccttttttgcggcattttgccttcctgtttttgctcacccagaaacgctggtgaaagtaaaagatgctgaagatcagttgggtgcacgagtgggttacatcgaactggatctcaacagcggtaagatccttgagagttttcgccccgaagaacgttttccaatgatgagcacttttaaagttctgctatgtggcgcggtattatcccgtgttgacgccgggcaagagcaactcggtcgccgcatacactattctcagaatgacttggttgagtactcaccagtcacagaaaagcatcttacggatggcatgacagtaagagaattatgcagtgctgccataaccatgagtgataacactgcggccaacttacttctgacaacgatcggaggaccgaaggagctaaccgcttttttgcacaacatgggggatcatgtaactcgccttgatcgttgggaaccggagctgaatgaagccataccaaacgacgagcgtgacaccacgatgcctgtagcaatggcaacaacgttgcgcaaactattaactggcgaactacttactctagcttcccggcaacaattaatagactggatggaggcggataaagttgcaggaccacttctgcgctcggcccttccggctggctggtttattgctgataaatctggagccggtgagcgtgggtctcgcggtatcattgcagcactggggccagatggtaagccctcccgtatcgtagttatctacacgacgggcagtcaggcaactatggatgaacgaaatagacagatcgctgagataggtgcctcactgattaagcattggtaactgtcagaccaagtttactcatatatactttagattgatttaaaacttcatttttaatttaaaaggatctaggtgaagatcctttttgataatctcatgaccaaaatcccttaacgtgagttttcgttccactgagcgtcagaccccgtagaaaagatcaaaggatcttcttgagatcctttttttctgcgcgtaatctgctgcttgcaaacaaaaaaaccaccgctaccagcggtggtttgtttgccggatcaagagctaccaactctttttccgaaggtaactggcttcagcagagcgcagataccaaatactgtccttctagtgtagccgtagttaggccaccacttcaagaactctgtagcaccgcctacatacctcgctctgctaatcctgttaccagtggctgctgccagtggcgataagtcgtgtcttaccgggttggactcaagacgatagttaccggataaggcgcagcggtcgggctgaacggggggttcgtgcacacagcccagcttggagcgaacgacctacaccgaactgagatacctacagcgtgagcattgagaaagcgccacgcttcccgaagggagaaaggcggacaggtatccggtaagcggcagggtcggaacaggagagcgcacgagggagcttccaggggggaacgcctggtatctttatagtcctgtcgggtttcgccacctctgacttgagcgtcgatttttgtgatgctcgtcaggggggccgagcctatggaaaaacgccagcaacgcggcctttttacggttcctggccttttgctggccttttgctcacatgttctttcctgcgttatcccctgattctgtggataaccgtattaccgcctttgagtgagctgataccgctcgccgcagccgaacgaccgagcgcagcgagtcagtgagcgaggaagcggaagagcgcccaatacgcaaaccgcctctccccgcgcgttggccgattcattaatgcagctggcacgacaggtttcccgactggaaagcgggcagtgagcgcaacgcaattaatgtgagttacctcactcattaggcaccccaggctttacactttatgcttccggctcctatgttgtgtggaattgtgagcggataacaatttcacacaggaaacagctatgaccatgattacgccaagctcggaattaaccctcactaaagggaacaaaagctggctagt

SEQ ID NO: 73 - DNA, 5009 bp, artificial
  modified vector pYD1Nhe
acggattagaagccgccgagcgggtgacagccctccgaaggaagactctcctccgtgcgtcctcgtcttcaccggtcgcgttcctgaaacgcagatgtgcctcgcgccgcactgctccgaacaataaagattctacaatactagcttttatggttatgaagaggaaaaattggcagtaacctggccccacaaaccttcaaatgaacgaatcaaattaacaaccataggatgataatgcgattagttttttagccttatttctggggtaattaatcagcgaagcgatgatttttgatctattaacagatatataaatgcaaaaactgcataaccactttaactaatactttcaacattttcggtttgtattacttcttattcaaatgtaataaaagtatcaacaaaaaattgttaatatacctctatactttaacgtcaaggagaaaaaaccccggatcggactactagcagctgtaatacgactcactatagggaatattaagctaattctacttcatacattttcaattaagatgcagttacttcgctgtttttcaatattttctgttattgcttcagtgctagcacaggaactgacaactatatgcgagcaaatcccctcaccaactttagaatcgacgccgtactctttgtcaacgactactattttggccaacgggaaggcaatgcaaggagtttttgaatattacaaatcagtaacgtttgtcagtaattgcggttctcacccctcaacaactagcaaaggcagccccataaacacacagtatgtttttaagcttctgcaggctagtggtggtggtggttctggtggtggtggttctggtggtggtggttctgctagcatgactggtggacagcaaatgggtcgggatctgtacgacgatgacgataaggtaccaggatccagtgtggtggaattctgcagatatccagcacagtggcggccgctcgagtctagagggcccttcgaaggtaagcctatccctaaccctctcctcggtctcgattctacgcgtaccggtcatcatcaccatcaccattgagtttaaacccgctgatctgataacaacagtgtagatgtaacaaaatcgactttgttcccactgtacttttagctcgtacaaaatacaatatacttttcatttctccgtaaacaacatgttttcccatgtaatatccttttctatttttcgttccgttaccaactttacacatactttatatagctattcacttctatacactaaaaaactaagacaattttaattttgctgcctgccatatttcaatttgttataaattcctataatttatcctattagtagctaaaaaaagatgaatgtgaatcgaatcctaagagaattgggcaagtgcacaaacaatacttaaataaatactactcagtaataacctatttcttagcatttttgacgaaatttgctattttgttagagtcttttacaccatttgtctccacacctccgcttacatcaacaccaataacgccatttaatctaagcgcatcaccaacattttctggcgtcagtccaccagctaacataaaatgtaagctctcggggctctcttgccttccaacccagtcagaaatcgagttccaatccaaaagttcacctgtcccacctgcttctgaatcaaacaagggaataaacgaatgaggtttctgtgaagctgcactgagtagtatgttgcagtcttttggaaatacgagtcttttaataactggcaaaccgaggaactcttggtattcttgccacgactcatctccgtgcagttggacgatatcaatgccgtaatcattgaccagagccaaaacatcctccttaggttgattacgaaacacgccaaccaagtatttcggagtgcctgaactatttttatatgcttttacaagacttgaaattttccttgcaataaccgggtcaattgttctctttctattgggcacacatataatacccagcaagtcagcatcggaatctagagcacattctgcggcctctgtgctctgcaagccgcaaactttcaccaatggaccagaactacctgtgaaattaataacagacatactccaagctgcctttgtgtgcttaatcacgtatactcacgtgctcaatagtcaccaatgccctccctcttggccctctccttttcttttttcgaccgaatttcttgaagacgaaagggcctcgtgatacgcctatttttataggttaatgtcatgataataatggtttcttaggacggatcgcttgcctgtaacttacacgcgcctcgtatcttttaatgatggaataatttgggaatttactctgtgtttatttatttttatgttttgtatttggattttagaaagtaaataaagaaggtagaagagttacggaatgaagaaaaaaaaataaacaaaggtttaaaaaatttcaacaaaaagcgtactttacatatatatttattagacaagaaaagcagattaaatagatatacattcgattaacgataagtaaaatgtaaaatcacaggattttcgtgtgtggtcttctacacagacaagatgaaacaattcggcattaatacctgagagcaggaagagcaagataaaaggtagtatttgttggcgatccccctagagtcttttacatcttcggaaaacaaaaactattttttctttaatttctttttttactttctatttttaatttatatatttatattaaaaaatttaaattataattatttttatagcacgtgatgaaaaggacccaggtggcacttttcggggaaatgtgcgcggaacccctatttgtttatttttctaaatacattcaaatatgtatccgctcatgagacaataaccctgataaatgcttcaataatattgaaaaaggaagagtatgagtattcaacatttccgtgtcgcccttattcccttttttgcggcattttgccttcctgtttttgctcacccagaaacgctggtgaaagtaaaagatgctgaagatcagttgggtgcacgagtgggttacatcgaactggatctcaacagcggtaagatccttgagagttttcgccccgaagaacgttttccaatgatgagcacttttaaagttctgctatgtggcgcggtattatcccgtgttgacgccgggcaagagcaactcggtcgccgcatacactattctcagaatgacttggttgagtactcaccagtcacagaaaagcatcttacggatggcatgacagtaagagaattatgcagtgctgccataaccatgagtgataacactgcggccaacttacttctgacaacgatcggaggaccgaaggagctaaccgcttttttgcacaacatgggggatcatgtaactcgccttgatcgttgggaaccggagctgaatgaagccataccaaacgacgagcgtgacaccacgatgcctgtagcaatggcaacaacgttgcgcaaactattaactggcgaactacttactctagcttcccggcaacaattaatagactggatggaggcggataaagttgcaggaccacttctgcgctcggcccttccggctggctggtttattgctgataaatctggagccggtgagcgtgggtctcgcggtatcattgcagcactggggccagatggtaagccctcccgtatcgtagttatctacacgacgggcagtcaggcaactatggatgaacgaaatagacagatcgctgagataggtgcctcactgattaagcattggtaactgtcagaccaagtttactcatatatactttagattgatttaaaacttcatttttaatttaaaaggatctaggtgaagatcctttttgataatctcatgaccaaaatcccttaacgtgagttttcgttccactgagcgtcagaccccgtagaaaagatcaaaggatcttcttgagatcctttttttctgcgcgtaatctgctgcttgcaaacaaaaaaaccaccgctaccagcggtggtttgtttgccggatcaagagctaccaactctttttccgaaggtaactggcttcagcagagcgcagataccaaatactgtccttctagtgtagccgtagttaggccaccacttcaagaactctgtagcaccgcctacatacctcgctctgctaatcctgttaccagtggctgctgccagtggcgataagtcgtgtcttaccgggttggactcaagacgatagttaccggataaggcgcagcggtcgggctgaacggggggttcgtgcacacagcccagcttggagcgaacgacctacaccgaactgagatacctacagcgtgagcattgagaaagcgccacgcttcccgaagggagaaaggcggacaggtatccggtaagcggcagggtcggaacaggagagcgcacgagggagcttccaggggggaacgcctggtatctttatagtcctgtcgggtttcgccacctctgacttgagcgtcgatttttgtgatgctcgtcaggggggccgagcctatggaaaaacgccagcaacgcggcctttttacggttcctggccttttgctggccttttgctcacatgttctttcctgcgttatcccctgattctgtggataaccgtattaccgcctttgagtgagctgataccgctcgccgcagccgaacgaccgagcgcagcgagtcagtgagcgaggaagcggaagagcgcccaatacgcaaaccgcctctccccgcgcgttggccgattcattaatgcagctggcacgacaggtttcccgactggaaagcgggcagtgagcgcaacgcaattaatgtgagttacctcactcattaggcaccccaggctttacactttatgcttccggctcctatgttgtgtggaattgtgagcggataacaatttcacacaggaaacagctatgaccatgattacgccaagctcggaattaaccctcactaaagggaacaaaagctggctagt

SEQ ID NO: 74 - DNA, 4605 bp, artificial
  vector pYD1lnk
acggattagaagccgccgagcgggtgacagccctccgaaggaagactctcctccgtgcgtcctcgtcttcaccggtcgcgttcctgaaacgcagatgtgcctcgcgccgcactgctccgaacaataaagattctacaatactagcttttatggttatgaagaggaaaaattggcagtaacctggccccacaaaccttcaaatgaacgaatcaaattaacaaccataggatgataatgcgattagttttttagccttatttctggggtaattaatcagcgaagcgatgatttttgatctattaacagatatataaatgcaaaaactgcataaccactttaactaatactttcaacattttcggtttgtattacttcttattcaaatgtaataaaagtatcaacaaaaaattgttaatatacctctatactttaacgtcaaggagaaaaaaccccggatcggactactagcagctgtaatacgactcactatagggaatattaagctaattctacttcatacattttcaattaagatgcagttacttcgctgtttttcaatattttctgttattgcttcagtgctagccgctggggccatggttactgattggcgcgccggatccttcagactctgcagaattcggccgcgtacttaattaagtttaaacccgctgatctgataacaacagtgtagatgtaacaaaatcgactttgttcccactgtacttttagctcgtacaaaatacaatatacttttcatttctccgtaaacaacatgttttcccatgtaatatccttttctatttttcgttccgttaccaactttacacatactttatatagctattcacttctatacactaaaaaactaagacaattttaattttgctgcctgccatatttcaatttgttataaattcctataatttatcctattagtagctaaaaaaagatgaatgtgaatcgaatcctaagagaattgggcaagtgcacaaacaatacttaaataaatactactcagtaataacctatttcttagcatttttgacgaaatttgctattttgttagagtcttttacaccatttgtctccacacctccgcttacatcaacaccaataacgccatttaatctaagcgcatcaccaacattttctggcgtcagtccaccagctaacataaaatgtaagctctcggggctctcttgccttccaacccagtcagaaatcgagttccaatccaaaagttcacctgtcccacctgcttctgaatcaaacaagggaataaacgaatgaggtttctgtgaagctgcactgagtagtatgttgcagtcttttggaaatacgagtcttttaataactggcaaaccgaggaactcttggtattcttgccacgactcatctccgtgcagttggacgatatcaatgccgtaatcattgaccagagccaaaacatcctccttaggttgattacgaaacacgccaaccaagtatttcggagtgcctgaactatttttatatgcttttacaagacttgaaattttccttgcaataaccgggtcaattgttctctttctattgggcacacatataatacccagcaagtcagcatcggaatctagagcacattctgcggcctctgtgctctgcaagccgcaaactttcaccaatggaccagaactacctgtgaaattaataacagacatactccaagctgcctttgtgtgcttaatcacgtatactcacgtgctcaatagtcaccaatgccctccctcttggccctctccttttcttttttcgaccgaatttcttgaagacgaaagggcctcgtgatacgcctatttttataggttaatgtcatgataataatggtttcttaggacggatcgcttgcctgtaacttacacgcgcctcgtatcttttaatgatggaataatttgggaatttactctgtgtttatttatttttatgttttgtatttggattttagaaagtaaataaagaaggtagaagagttacggaatgaagaaaaaaaaataaacaaaggtttaaaaaatttcaacaaaaagcgtactttacatatatatttattagacaagaaaagcagattaaatagatatacattcgattaacgataagtaaaatgtaaaatcacaggattttcgtgtgtggtcttctacacagacaagatgaaacaattcggcattaatacctgagagcaggaagagcaagataaaaggtagtatttgttggcgatccccctagagtcttttacatcttcggaaaacaaaaactattttttctttaatttctttttttactttctatttttaatttatatatttatattaaaaaatttaaattataattatttttatagcacgtgatgaaaaggacccaggtggcacttttcggggaaatgtgcgcggaacccctatttgtttatttttctaaatacattcaaatatgtatccgctcatgagacaataaccctgataaatgcttcaataatattgaaaaaggaagagtatgagtattcaacatttccgtgtcgcccttattcccttttttgcggcattttgccttcctgtttttgctcacccagaaacgctggtgaaagtaaaagatgctgaagatcagttgggtgcacgagtgggttacatcgaactggatctcaacagcggtaagatccttgagagttttcgccccgaagaacgttttccaatgatgagcacttttaaagttctgctatgtggcgcggtattatcccgtgttgacgccgggcaagagcaactcggtcgccgcatacactattctcagaatgacttggttgagtactcaccagtcacagaaaagcatcttacggatggcatgacagtaagagaattatgcagtgctgccataaccatgagtgataacactgcggccaacttacttctgacaacgatcggaggaccgaaggagctaaccgcttttttgcacaacatgggggatcatgtaactcgccttgatcgttgggaaccggagctgaatgaagccataccaaacgacgagcgtgacaccacgatgcctgtagcaatggcaacaacgttgcgcaaactattaactggcgaactacttactctagcttcccggcaacaattaatagactggatggaggcggataaagttgcaggaccacttctgcgctcggcccttccggctggctggtttattgctgataaatctggagccggtgagcgtgggtctcgcggtatcattgcagcactggggccagatggtaagccctcccgtatcgtagttatctacacgacgggcagtcaggcaactatggatgaacgaaatagacagatcgctgagataggtgcctcactgattaagcattggtaactgtcagaccaagtttactcatatatactttagattgatttaaaacttcatttttaatttaaaaggatctaggtgaagatcctttttgataatctcatgaccaaaatcccttaacgtgagttttcgttccactgagcgtcagaccccgtagaaaagatcaaaggatcttcttgagatcctttttttctgcgcgtaatctgctgcttgcaaacaaaaaaaccaccgctaccagcggtggtttgtttgccggatcaagagctaccaactctttttccgaaggtaactggcttcagcagagcgcagataccaaatactgtccttctagtgtagccgtagttaggccaccacttcaagaactctgtagcaccgcctacatacctcgctctgctaatcctgttaccagtggctgctgccagtggcgataagtcgtgtcttaccgggttggactcaagacgatagttaccggataaggcgcagcggtcgggctgaacggggggttcgtgcacacagcccagcttggagcgaacgacctacaccgaactgagatacctacagcgtgagcattgagaaagcgccacgcttcccgaagggagaaaggcggacaggtatccggtaagcggcagggtcggaacaggagagcgcacgagggagcttccaggggggaacgcctggtatctttatagtcctgtcgggtttcgccacctctgacttgagcgtcgatttttgtgatgctcgtcaggggggccgagcctatggaaaaacgccagcaacgcggcctttttacggttcctggccttttgctggccttttgctcacatgttctttcctgcgttatcccctgattctgtggataaccgtattaccgcctttgagtgagctgataccgctcgccgcagccgaacgaccgagcgcagcgagtcagtgagcgaggaagcggaagagcgcccaatacgcaaaccgcctctccccgcgcgttggccgattcattaatgcagctggcacgacaggtttcccgactggaaagcgggcagtgagcgcaacgcaattaatgtgagttacctcactcattaggcaccccaggctttacactttatgcttccggctcctatgttgtgtggaattgtgagcggataacaatttcacacaggaaacagctatgaccatgattacgccaagctcggaattaaccctcactaaagggaacaaaagctggctagt

SEQ ID NO: 75 - DNA, 4886 bp, artificial
  vector pYD1mata
acggattagaagccgccgagcgggtgacagccctccgaaggaagactctcctccgtgcgtcctcgtcttcaccggtcgcgttcctgaaacgcagatgtgcctcgcgccgcactgctccgaacaataaagattctacaatactagcttttatggttatgaagaggaaaaattggcagtaacctggccccacaaaccttcaaatgaacgaatcaaattaacaaccataggatgataatgcgattagttttttagccttatttctggggtaattaatcagcgaagcgatgatttttgatctattaacagatatataaatgcaaaaactgcataaccactttaactaatactttcaacattttcggtttgtattacttcttattcaaatgtaataaaagtatcaacaaaaaattgttaatatacctctatactttaacgtcaaggagaaaaaaccccggatcggactactagcagctgtaatacgactcactatagggaatattaagctaattctacttcatacattttcaattaagatgcagttacttcgctgtttttcaatattttctgttattgcttcagtgctagccgctggggccatggttactgattggcgcgccggatccgatgtaacaaaatcgactttgttcccactgtacttttagctcgtacaaaatacaatatacttttcatttctccgtaaacaacatgttttcccatgtaatatccttttctatttttcgttccgttaccaactttacacatactttatatagctattcacttctatacactaaaaaactaagacaattttaattttgctgcctgccatatttcaatttgttataaattcctataatttatcctattagtagctaaaaaaagatgaatgtgaatcgaatcctaagagaattgctgcagaattcggccgcgtacttaattaagtttaaacccgctgatctgataacaacagtgtagatgtaacaaaatcgactttgttcccactgtacttttagctcgtacaaaatacaatatacttttcatttctccgtaaacaacatgttttcccatgtaatatccttttctatttttcgttccgttaccaactttacacatactttatatagctattcacttctatacactaaaaaactaagacaattttaattttgctgcctgccatatttcaatttgttataaattcctataatttatcctattagtagctaaaaaaagatgaatgtgaatcgaatcctaagagaattgggcaagtgcacaaacaatacttaaataaatactactcagtaataacctatttcttagcatttttgacgaaatttgctattttgttagagtcttttacaccatttgtctccacacctccgcttacatcaacaccaataacgccatttaatctaagcgcatcaccaacattttctggcgtcagtccaccagctaacataaaatgtaagctctcggggctctcttgccttccaacccagtcagaaatcgagttccaatccaaaagttcacctgtcccacctgcttctgaatcaaacaagggaataaacgaatgaggtttctgtgaagctgcactgagtagtatgttgcagtcttttggaaatacgagtcttttaataactggcaaaccgaggaactcttggtattcttgccacgactcatctccgtgcagttggacgatatcaatgccgtaatcattgaccagagccaaaacatcctccttaggttgattacgaaacacgccaaccaagtatttcggagtgcctgaactatttttatatgcttttacaagacttgaaattttccttgcaataaccgggtcaattgttctctttctattgggcacacatataatacccagcaagtcagcatcggaatctagagcacattctgcggcctctgtgctctgcaagccgcaaactttcaccaatggaccagaactacctgtgaaattaataacagacatactccaagctgcctttgtgtgcttaatcacgtatactcacgtgctcaatagtcaccaatgccctccctcttggccctctccttttcttttttcgaccgaatttcttgaagacgaaagggcctcgtgatacgcctatttttataggttaatgtcatgataataatggtttcttaggacggatcgcttgcctgtaacttacacgcgcctcgtatcttttaatgatggaataatttgggaatttactctgtgtttatttatttttatgttttgtatttggattttagaaagtaaataaagaaggtagaagagttacggaatgaagaaaaaaaaataaacaaaggtttaaaaaatttcaacaaaaagcgtactttacatatatatttattagacaagaaaagcagattaaatagatatacattcgattaacgataagtaaaatgtaaaatcacaggattttcgtgtgtggtcttctacacagacaagatgaaacaattcggcattaatacctgagagcaggaagagcaagataaaaggtagtatttgttggcgatccccctagagtcttttacatcttcggaaaacaaaaactattttttctttaatttctttttttactttctatttttaatttatatatttatattaaaaaatttaaattataattatttttatagcacgtgatgaaaaggacccaggtggcacttttcggggaaatgtgcgcggaacccctatttgtttatttttctaaatacattcaaatatgtatccgctcatgagacaataaccctgataaatgcttcaataatattgaaaaaggaagagtatgagtattcaacatttccgtgtcgcccttattcccttttttgcggcattttgccttcctgtttttgctcacccagaaacgctggtgaaagtaaaagatgctgaagatcagttgggtgcacgagtgggttacatcgaactggatctcaacagcggtaagatccttgagagttttcgccccgaagaacgttttccaatgatgagcacttttaaagttctgctatgtggcgcggtattatcccgtgttgacgccgggcaagagcaactcggtcgccgcatacactattctcagaatgacttggttgagtactcaccagtcacagaaaagcatcttacggatggcatgacagtaagagaattatgcagtgctgccataaccatgagtgataacactgcggccaacttacttctgacaacgatcggaggaccgaaggagctaaccgcttttttgcacaacatgggggatcatgtaactcgccttgatcgttgggaaccggagctgaatgaagccataccaaacgacgagcgtgacaccacgatgcctgtagcaatggcaacaacgttgcgcaaactattaactggcgaactacttactctagcttcccggcaacaattaatagactggatggaggcggataaagttgcaggaccacttctgcgctcggcccttccggctggctggtttattgctgataaatctggagccggtgagcgtgggtctcgcggtatcattgcagcactggggccagatggtaagccctcccgtatcgtagttatctacacgacgggcagtcaggcaactatggatgaacgaaatagacagatcgctgagataggtgcctcactgattaagcattggtaactgtcagaccaagtttactcatatatactttagattgatttaaaacttcatttttaatttaaaaggatctaggtgaagatcctttttgataatctcatgaccaaaatcccttaacgtgagttttcgttccactgagcgtcagaccccgtagaaaagatcaaaggatcttcttgagatcctttttttctgcgcgtaatctgctgcttgcaaacaaaaaaaccaccgctaccagcggtggtttgtttgccggatcaagagctaccaactctttttccgaaggtaactggcttcagcagagcgcagataccaaatactgtccttctagtgtagccgtagttaggccaccacttcaagaactctgtagcaccgcctacatacctcgctctgctaatcctgttaccagtggctgctgccagtggcgataagtcgtgtcttaccgggttggactcaagacgatagttaccggataaggcgcagcggtcgggctgaacggggggttcgtgcacacagcccagcttggagcgaacgacctacaccgaactgagatacctacagcgtgagcattgagaaagcgccacgcttcccgaagggagaaaggcggacaggtatccggtaagcggcagggtcggaacaggagagcgcacgagggagcttccaggggggaacgcctggtatctttatagtcctgtcgggtttcgccacctctgacttgagcgtcgatttttgtgatgctcgtcaggggggccgagcctatggaaaaacgccagcaacgcggcctttttacggttcctggccttttgctggccttttgctcacatgttctttcctgcgttatcccctgattctgtggataaccgtattaccgcctttgagtgagctgataccgctcgccgcagccgaacgaccgagcgcagcgagtcagtgagcgaggaagcggaagagcgcccaatacgcaaaccgcctctccccgcgcgttggccgattcattaatgcagctggcacgacaggtttcccgactggaaagcgggcagtgagcgcaacgcaattaatgtgagttacctcactcattaggcaccccaggctttacactttatgcttccggctcctatgttgtgtggaattgtgagcggataacaatttcacacaggaaacagctatgaccatgattacgccaagctcggaattaaccctcactaaagggaacaaaagctggctagt

SEQ ID NO: 76 - DNA, 5801 bp, artificial
  vector pYD1gal
acggattagaagccgccgagcgggtgacagccctccgaaggaagactctcctccgtgcgtcctcgtcttcaccggtcgcgttcctgaaacgcagatgtgcctcgcgccgcactgctccgaacaataaagattctacaatactagcttttatggttatgaagaggaaaaattggcagtaacctggccccacaaaccttcaaatgaacgaatcaaattaacaaccataggatgataatgcgattagttttttagccttatttctggggtaattaatcagcgaagcgatgatttttgatctattaacagatatataaatgcaaaaactgcataaccactttaactaatactttcaacattttcggtttgtattacttcttattcaaatgtaataaaagtatcaacaaaaaattgttaatatacctctatactttaacgtcaaggagaaaaaaccccggatcggactactagcagctgtaatacgactcactatagggaatattaagctaattctacttcatacattttcaattaagatgcagttacttcgctgtttttcaatattttctgttattgcttcagtgctagccgctggggccatggttactgattggcgcgccggatccgatgtaacaaaatcgactttgttcccactgtacttttagctcgtacaaaatacaatatacttttcatttctccgtaaacaacatgttttcccatgtaatatccttttctatttttcgttccgttaccaactttacacatactttatatagctattcacttctatacactaaaaaactaagacaattttaattttgctgcctgccatatttcaatttgttataaattcctataatttatcctattagtagctaaaaaaagatgaatgtgaatcgaatcctaagagaattgctgcagaattcacggattagaagccgccgagcgggtgacagccctccgaaggaagactctcctccgtgcgtcctcgtcttcaccggtcgcgttcctgaaacgcagatgtgcctcgcgccgcactgctccgaacaataaagattctacaatactagcttttatggttatgaagaggaaaaattggcagtaacctggccccacaaaccttcaaatgaacgaatcaaattaacaaccataggatgataatgcgattagttttttagccttatttctggggtaattaatcagcgaagcgatgatttttgatctattaacagatatataaatgcaaaaactgcataaccactttaactaatactttcaacattttcggtttgtattacttcttattcaaatgtaataaaagtatcaacaaaaaattgttaatatacctctatactttaacgtcaaggagaaaaaaccccggatcggactactagcagctgtaatacgactcactatagggaatattaagctaattctacttcatacattttcaattaagatgcagttacttcgctgtttttcaatattttctgttattgcttcagttttagcacaggaactgacaactatatgcgagcaaatcccctcaccaactttagaatcgacgccgtactctttgtcaacgactactattttggccaacgggaaggcaatgcaaggagtttttgaatattacaaatcagtaacgtttgtcagtaattgcggttctcacccctcaacaactagcaaaggcagccccataaacacacagtatgtttttaagcttctgcaggctagtggtggtggtggttctggtggtggtggttctggtggtggtggttctgctagcatgactggtggccagcaaggcctaattctgatgcggccgcacatcatcaccatcaccattgattaattaagtttaaacccgctgatctgataacaacagtgtagatgtaacaaaatcgactttgttcccactgtacttttagctcgtacaaaatacaatatacttttcatttctccgtaaacaacatgttttcccatgtaatatccttttctatttttcgttccgttaccaactttacacatactttatatagctattcacttctatacactaaaaaactaagacaattttaattttgctgcctgccatatttcaatttgttataaattcctataatttatcctattagtagctaaaaaaagatgaatgtgaatcgaatcctaagagaattgggcaagtgcacaaacaatacttaaataaatactactcagtaataacctatttcttagcatttttgacgaaatttgctattttgttagagtcttttacaccatttgtctccacacctccgcttacatcaacaccaataacgccatttaatctaagcgcatcaccaacattttctggcgtcagtccaccagctaacataaaatgtaagctctcggggctctcttgccttccaacccagtcagaaatcgagttccaatccaaaagttcacctgtcccacctgcttctgaatcaaacaagggaataaacgaatgaggtttctgtgaagctgcactgagtagtatgttgcagtcttttggaaatacgagtcttttaataactggcaaaccgaggaactcttggtattcttgccacgactcatctccgtgcagttggacgatatcaatgccgtaatcattgaccagagccaaaacatcctccttaggttgattacgaaacacgccaaccaagtatttcggagtgcctgaactatttttatatgcttttacaagacttgaaattttccttgcaataaccgggtcaattgttctctttctattgggcacacatataatacccagcaagtcagcatcggaatctagagcacattctgcggcctctgtgctctgcaagccgcaaactttcaccaatggaccagaactacctgtgaaattaataacagacatactccaagctgcctttgtgtgcttaatcacgtatactcacgtgctcaatagtcaccaatgccctccctcttggccctctccttttcttttttcgaccgaatttcttgaagacgaaagggcctcgtgatacgcctatttttataggttaatgtcatgataataatggtttcttaggacggatcgcttgcctgtaacttacacgcgcctcgtatcttttaatgatggaataatttgggaatttactctgtgtttatttatttttatgttttgtatttggattttagaaagtaaataaagaaggtagaagagttacggaatgaagaaaaaaaaataaacaaaggtttaaaaaatttcaacaaaaagcgtactttacatatatatttattagacaagaaaagcagattaaatagatatacattcgattaacgataagtaaaatgtaaaatcacaggattttcgtgtgtggtcttctacacagacaagatgaaacaattcggcattaatacctgagagcaggaagagcaagataaaaggtagtatttgttggcgatccccctagagtcttttacatcttcggaaaacaaaaactattttttctttaatttctttttttactttctatttttaatttatatatttatattaaaaaatttaaattataattatttttatagcacgtgatgaaaaggacccaggtggcacttttcggggaaatgtgcgcggaacccctatttgtttatttttctaaatacattcaaatatgtatccgctcatgagacaataaccctgataaatgcttcaataatattgaaaaaggaagagtatgagtattcaacatttccgtgtcgcccttattcccttttttgcggcattttgccttcctgtttttgctcacccagaaacgctggtgaaagtaaaagatgctgaagatcagttgggtgcacgagtgggttacatcgaactggatctcaacagcggtaagatccttgagagttttcgccccgaagaacgttttccaatgatgagcacttttaaagttctgctatgtggcgcggtattatcccgtgttgacgccgggcaagagcaactcggtcgccgcatacactattctcagaatgacttggttgagtactcaccagtcacagaaaagcatcttacggatggcatgacagtaagagaattatgcagtgctgccataaccatgagtgataacactgcggccaacttacttctgacaacgatcggaggaccgaaggagctaaccgcttttttgcacaacatgggggatcatgtaactcgccttgatcgttgggaaccggagctgaatgaagccataccaaacgacgagcgtgacaccacgatgcctgtagcaatggcaacaacgttgcgcaaactattaactggcgaactacttactctagcttcccggcaacaattaatagactggatggaggcggataaagttgcaggaccacttctgcgctcggcccttccggctggctggtttattgctgataaatctggagccggtgagcgtgggtctcgcggtatcattgcagcactggggccagatggtaagccctcccgtatcgtagttatctacacgacgggcagtcaggcaactatggatgaacgaaatagacagatcgctgagataggtgcctcactgattaagcattggtaactgtcagaccaagtttactcatatatactttagattgatttaaaacttcatttttaatttaaaaggatctaggtgaagatcctttttgataatctcatgaccaaaatcccttaacgtgagttttcgttccactgagcgtcagaccccgtagaaaagatcaaaggatcttcttgagatcctttttttctgcgcgtaatctgctgcttgcaaacaaaaaaaccaccgctaccagcggtggtttgtttgccggatcaagagctaccaactctttttccgaaggtaactggcttcagcagagcgcagataccaaatactgtccttctagtgtagccgtagttaggccaccacttcaagaactctgtagcaccgcctacatacctcgctctgctaatcctgttaccagtggctgctgccagtggcgataagtcgtgtcttaccgggttggactcaagacgatagttaccggataaggcgcagcggtcgggctgaacggggggttcgtgcacacagcccagcttggagcgaacgacctacaccgaactgagatacctacagcgtgagcattgagaaagcgccacgcttcccgaagggagaaaggcggacaggtatccggtaagcggcagggtcggaacaggagagcgcacgagggagcttccaggggggaacgcctggtatctttatagtcctgtcgggtttcgccacctctgacttgagcgtcgatttttgtgatgctcgtcaggggggccgagcctatggaaaaacgccagcaacgcggcctttttacggttcctggccttttgctggccttttgctcacatgttctttcctgcgttatcccctgattctgtggataaccgtattaccgcctttgagtgagctgataccgctcgccgcagccgaacgaccgagcgcagcgagtcagtgagcgaggaagcggaagagcgcccaatacgcaaaccgcctctccccgcgcgttggccgattcattaatgcagctggcacgacaggtttcccgactggaaagcgggcagtgagcgcaacgcaattaatgtgagttacctcactcattaggcaccccaggctttacactttatgcttccggctcctatgttgtgtggaattgtgagcggataacaatttcacacaggaaacagctatgaccatgattacgccaagctcggaattaaccctcactaaagggaacaaaagctggctagt

SEQ ID NO: 77 - DNA, 692 bp, artificial
  4D5H
ggccagcaaggccaagaggttcaactagtggagtctggcggtggcctggtgcagccagggggctcactccgtttgtcctgtgcagcttctggcttcaacattaaagacacctatatacactgggtgcgtcaggccccgggtaagggcctggaatgggttgcaaggatttatcctacgaatggttatactagatatgccgatagcgtcaagggccgtttcactataagcgcagacacatccaaaaacacagcctacctgcagatgaacagcctgcgtgctgaggacactgccgtctattattgttctagatggggaggggacggcttctatgctatggactactggggtcaaggaaccctggtcaccgtctcctcggctagcaccaagggccccagcgtgttccctctggcccccagctccaagagcacctccggcggcaccgccgccctgggctgcctggtgaaggattacttcccagagcccgtgaccgtgagctggaacagcggcgccctgaccagcggcgtgcacacctttcccgccgtgctgcagtccagcggcctgtactccctgagcagcgtggtgaccgtgcccagcagcagcctgggcacccagacctacatctgcaatgtgaaccacaagcccagcaataccaaggtggataagaaggtggagcccaagagctgcgcggccgc

SEQ ID NO: 78 - DNA, 661 bp, artificial
  4D5L
ccatggcggatatccagatgacccagtccccgagctccctgtccgcctctgtgggcgatagggtcaccatcacctgccgtgccagtcaggatgtgaatactgctgtagcctggtatcaacagaaaccaggaaaagctccgaaactactgatttactcggcatccttcctctactctggagtcccttctcgcttctctggatccagatctgggacggatttcactctgaccatcagcagtctgcagccggaagacttcgcaacttattactgtcagcaacattatactactcctcccacgttcggacagggtaccaaggtggagatcaaacgtacggtggcggcgccatctgtcttcatcttcccgccatctgatgagcagcttaagtctggaactgcctctgttgtgtgcctgctgaataacttctatcccagagaggccaaagtacagtggaaggtggataacgccctccaatcgggtaactcccaggagagtgtcacagagcaggacagcaaggacagcacctacagcctcagcagcaccctgacgctgagcaaagcagactacgagaaacacaaagtctacgcctgcgaagtcacccatcagggcctgagctcgcccgtcacaaagagcttcaacaggggagagtgttgaggcgcgcc

SEQ ID NO: 79 - DNA, 6468 bp, artificial
  vector pYD4D5hc
acggattagaagccgccgagcgggtgacagccctccgaaggaagactctcctccgtgcgtcctcgtcttcaccggtcgcgttcctgaaacgcagatgtgcctcgcgccgcactgctccgaacaataaagattctacaatactagcttttatggttatgaagaggaaaaattggcagtaacctggccccacaaaccttcaaatgaacgaatcaaattaacaaccataggatgataatgcgattagttttttagccttatttctggggtaattaatcagcgaagcgatgatttttgatctattaacagatatataaatgcaaaaactgcataaccactttaactaatactttcaacattttcggtttgtattacttcttattcaaatgtaataaaagtatcaacaaaaaattgttaatatacctctatactttaacgtcaaggagaaaaaaccccggatcggactactagcagctgtaatacgactcactatagggaatattaagctaattctacttcatacattttcaattaagatgcagttacttcgctgtttttcaatattttctgttattgcttcagtgctagccgctggggccatggttactgattggcgcgccggatccgatgtaacaaaatcgactttgttcccactgtacttttagctcgtacaaaatacaatatacttttcatttctccgtaaacaacatgttttcccatgtaatatccttttctatttttcgttccgttaccaactttacacatactttatatagctattcacttctatacactaaaaaactaagacaattttaattttgctgcctgccatatttcaatttgttataaattcctataatttatcctattagtagctaaaaaaagatgaatgtgaatcgaatcctaagagaattgctgcagaattcacggattagaagccgccgagcgggtgacagccctccgaaggaagactctcctccgtgcgtcctcgtcttcaccggtcgcgttcctgaaacgcagatgtgcctcgcgccgcactgctccgaacaataaagattctacaatactagcttttatggttatgaagaggaaaaattggcagtaacctggccccacaaaccttcaaatgaacgaatcaaattaacaaccataggatgataatgcgattagttttttagccttatttctggggtaattaatcagcgaagcgatgatttttgatctattaacagatatataaatgcaaaaactgcataaccactttaactaatactttcaacattttcggtttgtattacttcttattcaaatgtaataaaagtatcaacaaaaaattgttaatatacctctatactttaacgtcaaggagaaaaaaccccggatcggactactagcagctgtaatacgactcactatagggaatattaagctaattctacttcatacattttcaattaagatgcagttacttcgctgtttttcaatattttctgttattgcttcagttttagcacaggaactgacaactatatgcgagcaaatcccctcaccaactttagaatcgacgccgtactctttgtcaacgactactattttggccaacgggaaggcaatgcaaggagtttttgaatattacaaatcagtaacgtttgtcagtaattgcggttctcacccctcaacaactagcaaaggcagccccataaacacacagtatgtttttaagcttctgcaggctagtggtggtggtggttctggtggtggtggttctggtggtggtggttctgctagcatgactggtggccagcaaggccaaggttctgaggttcaactagtggagtctggcggtggcctggtgcagccagggggctcactccgtttgtcctgtgcagcttctggcttcaacattaaagacacctatatacactgggtgcgtcaggccccgggtaagggcctggaatgggttgcaaggatttatcctacgaatggttatactagatatgccgatagcgtcaagggccgtttcactataagcgcagacacatccaaaaacacagcctacctgcagatgaacagcctgcgtgctgaggacactgccgtctattattgttctagatggggaggggacggcttctatgctatggactactggggtcaaggaaccctggtcaccgtctcctcggctagcaccaagggccccagcgtgttccctctggcccccagctccaagagcacctccggcggcaccgccgccctgggctgcctggtgaaggattacttcccagagcccgtgaccgtgagctggaacagcggcgccctgaccagcggcgtgcacacctttcccgccgtgctgcagtccagcggcctgtactccctgagcagcgtggtgaccgtgcccagcagcagcctgggcacccagacctacatctgcaatgtgaaccacaagcccagcaataccaaggtggataagaaggtggagcccaagagctgcgcggccgcacatcatcaccatcaccattgattaattaagtttaaacccgctgatctgataacaacagtgtagatgtaacaaaatcgactttgttcccactgtacttttagctcgtacaaaatacaatatacttttcatttctccgtaaacaacatgttttcccatgtaatatccttttctatttttcgttccgttaccaactttacacatactttatatagctattcacttctatacactaaaaaactaagacaattttaattttgctgcctgccatatttcaatttgttataaattcctataatttatcctattagtagctaaaaaaagatgaatgtgaatcgaatcctaagagaattgggcaagtgcacaaacaatacttaaataaatactactcagtaataacctatttcttagcatttttgacgaaatttgctattttgttagagtcttttacaccatttgtctccacacctccgcttacatcaacaccaataacgccatttaatctaagcgcatcaccaacattttctggcgtcagtccaccagctaacataaaatgtaagctctcggggctctcttgccttccaacccagtcagaaatcgagttccaatccaaaagttcacctgtcccacctgcttctgaatcaaacaagggaataaacgaatgaggtttctgtgaagctgcactgagtagtatgttgcagtcttttggaaatacgagtcttttaataactggcaaaccgaggaactcttggtattcttgccacgactcatctccgtgcagttggacgatatcaatgccgtaatcattgaccagagccaaaacatcctccttaggttgattacgaaacacgccaaccaagtatttcggagtgcctgaactatttttatatgcttttacaagacttgaaattttccttgcaataaccgggtcaattgttctctttctattgggcacacatataatacccagcaagtcagcatcggaatctagagcacattctgcggcctctgtgctctgcaagccgcaaactttcaccaatggaccagaactacctgtgaaattaataacagacatactccaagctgcctttgtgtgcttaatcacgtatactcacgtgctcaatagtcaccaatgccctccctcttggccctctccttttcttttttcgaccgaatttcttgaagacgaaagggcctcgtgatacgcctatttttataggttaatgtcatgataataatggtttcttaggacggatcgcttgcctgtaacttacacgcgcctcgtatcttttaatgatggaataatttgggaatttactctgtgtttatttatttttatgttttgtatttggattttagaaagtaaataaagaaggtagaagagttacggaatgaagaaaaaaaaataaacaaaggtttaaaaaatttcaacaaaaagcgtactttacatatatatttattagacaagaaaagcagattaaatagatatacattcgattaacgataagtaaaatgtaaaatcacaggattttcgtgtgtggtcttctacacagacaagatgaaacaattcggcattaatacctgagagcaggaagagcaagataaaaggtagtatttgttggcgatccccctagagtcttttacatcttcggaaaacaaaaactattttttctttaatttctttttttactttctatttttaatttatatatttatattaaaaaatttaaattataattatttttatagcacgtgatgaaaaggacccaggtggcacttttcggggaaatgtgcgcggaacccctatttgtttatttttctaaatacattcaaatatgtatccgctcatgagacaataaccctgataaatgcttcaataatattgaaaaaggaagagtatgagtattcaacatttccgtgtcgcccttattcccttttttgcggcattttgccttcctgtttttgctcacccagaaacgctggtgaaagtaaaagatgctgaagatcagttgggtgcacgagtgggttacatcgaactggatctcaacagcggtaagatccttgagagttttcgccccgaagaacgttttccaatgatgagcacttttaaagttctgctatgtggcgcggtattatcccgtgttgacgccgggcaagagcaactcggtcgccgcatacactattctcagaatgacttggttgagtactcaccagtcacagaaaagcatcttacggatggcatgacagtaagagaattatgcagtgctgccataaccatgagtgataacactgcggccaacttacttctgacaacgatcggaggaccgaaggagctaaccgcttttttgcacaacatgggggatcatgtaactcgccttgatcgttgggaaccggagctgaatgaagccataccaaacgacgagcgtgacaccacgatgcctgtagcaatggcaacaacgttgcgcaaactattaactggcgaactacttactctagcttcccggcaacaattaatagactggatggaggcggataaagttgcaggaccacttctgcgctcggcccttccggctggctggtttattgctgataaatctggagccggtgagcgtgggtctcgcggtatcattgcagcactggggccagatggtaagccctcccgtatcgtagttatctacacgacgggcagtcaggcaactatggatgaacgaaatagacagatcgctgagataggtgcctcactgattaagcattggtaactgtcagaccaagtttactcatatatactttagattgatttaaaacttcatttttaatttaaaaggatctaggtgaagatcctttttgataatctcatgaccaaaatcccttaacgtgagttttcgttccactgagcgtcagaccccgtagaaaagatcaaaggatcttcttgagatcctttttttctgcgcgtaatctgctgcttgcaaacaaaaaaaccaccgctaccagcggtggtttgtttgccggatcaagagctaccaactctttttccgaaggtaactggcttcagcagagcgcagataccaaatactgtccttctagtgtagccgtagttaggccaccacttcaagaactctgtagcaccgcctacatacctcgctctgctaatcctgttaccagtggctgctgccagtggcgataagtcgtgtcttaccgggttggactcaagacgatagttaccggataaggcgcagcggtcgggctgaacggggggttcgtgcacacagcccagcttggagcgaacgacctacaccgaactgagatacctacagcgtgagcattgagaaagcgccacgcttcccgaagggagaaaggcggacaggtatccggtaagcggcagggtcggaacaggagagcgcacgagggagcttccaggggggaacgcctggtatctttatagtcctgtcgggtttcgccacctctgacttgagcgtcgatttttgtgatgctcgtcaggggggccgagcctatggaaaaacgccagcaacgcggcctttttacggttcctggccttttgctggccttttgctcacatgttctttcctgcgttatcccctgattctgtggataaccgtattaccgcctttgagtgagctgataccgctcgccgcagccgaacgaccgagcgcagcgagtcagtgagcgaggaagcggaagagcgcccaatacgcaaaccgcctctccccgcgcgttggccgattcattaatgcagctggcacgacaggtttcccgactggaaagcgggcagtgagcgcaacgcaattaatgtgagttacctcactcattaggcaccccaggctttacactttatgcttccggctcctatgttgtgtggaattgtgagcggataacaatttcacacaggaaacagctatgaccatgattacgccaagctcggaattaaccctcactaaagggaacaaaagctggctagt

SEQ ID NO: 80 - protein, 223 aa, artificial
  4D5hp
EVQLVESGGGLVQPGGSLRLSCAASGFNIKDTYIHWVRQAPGKGLEWVARIYPTNGYTRYADSVKGRFTISADTSKNTAYLQMNSLRAEDTAVYYCSRWGGDGFYAMDYWGQGTLVTVSSASTKGPSVFPLAPSSKSTSGGTAALGCLVKDYFPEPVTVSWNSGALTSGVHTFPAVLQSSGLYSLSSVVTVPSSSLGTQTYICNVNHKPSNTKVDKKVEPKSC

SEQ ID NO: 81 - DNA, 7100 bp, artificial
  vector pYD4D5hl
acggattagaagccgccgagcgggtgacagccctccgaaggaagactctcctccgtgcgtcctcgtcttcaccggtcgcgttcctgaaacgcagatgtgcctcgcgccgcactgctccgaacaataaagattctacaatactagcttttatggttatgaagaggaaaaattggcagtaacctggccccacaaaccttcaaatgaacgaatcaaattaacaaccataggatgataatgcgattagttttttagccttatttctggggtaattaatcagcgaagcgatgatttttgatctattaacagatatataaatgcaaaaactgcataaccactttaactaatactttcaacattttcggtttgtattacttcttattcaaatgtaataaaagtatcaacaaaaaattgttaatatacctctatactttaacgtcaaggagaaaaaaccccggatcggactactagcagctgtaatacgactcactatagggaatattaagctaattctacttcatacattttcaattaagatgcagttacttcgctgtttttcaatattttctgttattgcttcagtgctagccgctggggccatggcggatatccagatgacccagtccccgagctccctgtccgcctctgtgggcgatagggtcaccatcacctgccgtgccagtcaggatgtgaatactgctgtagcctggtatcaacagaaaccaggaaaagctccgaaactactgatttactcggcatccttcctctactctggagtcccttctcgcttctctggatccagatctgggacggatttcactctgaccatcagcagtctgcagccggaagacttcgcaacttattactgtcagcaacattatactactcctcccacgttcggacagggtaccaaggtggagatcaaacgtacggtggcggcgccatctgtcttcatcttcccgccatctgatgagcagcttaagtctggaactgcctctgttgtgtgcctgctgaataacttctatcccagagaggccaaagtacagtggaaggtggataacgccctccaatcgggtaactcccaggagagtgtcacagagcaggacagcaaggacagcacctacagcctcagcagcaccctgacgctgagcaaagcagactacgagaaacacaaagtctacgcctgcgaagtcacccatcagggcctgagctcgcccgtcacaaagagcttcaacaggggagagtgttgaggcgcgccggatccgatgtaacaaaatcgactttgttcccactgtacttttagctcgtacaaaatacaatatacttttcatttctccgtaaacaacatgttttcccatgtaatatccttttctatttttcgttccgttaccaactttacacatactttatatagctattcacttctatacactaaaaaactaagacaattttaattttgctgcctgccatatttcaatttgttataaattcctataatttatcctattagtagctaaaaaaagatgaatgtgaatcgaatcctaagagaattgctgcagaattcacggattagaagccgccgagcgggtgacagccctccgaaggaagactctcctccgtgcgtcctcgtcttcaccggtcgcgttcctgaaacgcagatgtgcctcgcgccgcactgctccgaacaataaagattctacaatactagcttttatggttatgaagaggaaaaattggcagtaacctggccccacaaaccttcaaatgaacgaatcaaattaacaaccataggatgataatgcgattagttttttagccttatttctggggtaattaatcagcgaagcgatgatttttgatctattaacagatatataaatgcaaaaactgcataaccactttaactaatactttcaacattttcggtttgtattacttcttattcaaatgtaataaaagtatcaacaaaaaattgttaatatacctctatactttaacgtcaaggagaaaaaaccccggatcggactactagcagctgtaatacgactcactatagggaatattaagctaattctacttcatacattttcaattaagatgcagttacttcgctgtttttcaatattttctgttattgcttcagttttagcacaggaactgacaactatatgcgagcaaatcccctcaccaactttagaatcgacgccgtactctttgtcaacgactactattttggccaacgggaaggcaatgcaaggagtttttgaatattacaaatcagtaacgtttgtcagtaattgcggttctcacccctcaacaactagcaaaggcagccccataaacacacagtatgtttttaagcttctgcaggctagtggtggtggtggttctggtggtggtggttctggtggtggtggttctgctagcatgactggtggccagcaaggccaagaggttcaactagtggagtctggcggtggcctggtgcagccagggggctcactccgtttgtcctgtgcagcttctggcttcaacattaaagacacctatatacactgggtgcgtcaggccccgggtaagggcctggaatgggttgcaaggatttatcctacgaatggttatactagatatgccgatagcgtcaagggccgtttcactataagcgcagacacatccaaaaacacagcctacctgcagatgaacagcctgcgtgctgaggacactgccgtctattattgttctagatggggaggggacggcttctatgctatggactactggggtcaaggaaccctggtcaccgtctcctcggctagcaccaagggccccagcgtgttccctctggcccccagctccaagagcacctccggcggcaccgccgccctgggctgcctggtgaaggattacttcccagagcccgtgaccgtgagctggaacagcggcgccctgaccagcggcgtgcacacctttcccgccgtgctgcagtccagcggcctgtactccctgagcagcgtggtgaccgtgcccagcagcagcctgggcacccagacctacatctgcaatgtgaaccacaagcccagcaataccaaggtggataagaaggtggagcccaagagctgcgcggccgcacatcatcaccatcaccattgattaattaagtttaaacccgctgatctgataacaacagtgtagatgtaacaaaatcgactttgttcccactgtacttttagctcgtacaaaatacaatatacttttcatttctccgtaaacaacatgttttcccatgtaatatccttttctatttttcgttccgttaccaactttacacatactttatatagctattcacttctatacactaaaaaactaagacaattttaattttgctgcctgccatatttcaatttgttataaattcctataatttatcctattagtagctaaaaaaagatgaatgtgaatcgaatcctaagagaattgggcaagtgcacaaacaatacttaaataaatactactcagtaataacctatttcttagcatttttgacgaaatttgctattttgttagagtcttttacaccatttgtctccacacctccgcttacatcaacaccaataacgccatttaatctaagcgcatcaccaacattttctggcgtcagtccaccagctaacataaaatgtaagctctcggggctctcttgccttccaacccagtcagaaatcgagttccaatccaaaagttcacctgtcccacctgcttctgaatcaaacaagggaataaacgaatgaggtttctgtgaagctgcactgagtagtatgttgcagtcttttggaaatacgagtcttttaataactggcaaaccgaggaactcttggtattcttgccacgactcatctccgtgcagttggacgatatcaatgccgtaatcattgaccagagccaaaacatcctccttaggttgattacgaaacacgccaaccaagtatttcggagtgcctgaactatttttatatgcttttacaagacttgaaattttccttgcaataaccgggtcaattgttctctttctattgggcacacatataatacccagcaagtcagcatcggaatctagagcacattctgcggcctctgtgctctgcaagccgcaaactttcaccaatggaccagaactacctgtgaaattaataacagacatactccaagctgcctttgtgtgcttaatcacgtatactcacgtgctcaatagtcaccaatgccctccctcttggccctctccttttcttttttcgaccgaatttcttgaagacgaaagggcctcgtgatacgcctatttttataggttaatgtcatgataataatggtttcttaggacggatcgcttgcctgtaacttacacgcgcctcgtatcttttaatgatggaataatttgggaatttactctgtgtttatttatttttatgttttgtatttggattttagaaagtaaataaagaaggtagaagagttacggaatgaagaaaaaaaaataaacaaaggtttaaaaaatttcaacaaaaagcgtactttacatatatatttattagacaagaaaagcagattaaatagatatacattcgattaacgataagtaaaatgtaaaatcacaggattttcgtgtgtggtcttctacacagacaagatgaaacaattcggcattaatacctgagagcaggaagagcaagataaaaggtagtatttgttggcgatccccctagagtcttttacatcttcggaaaacaaaaactattttttctttaatttctttttttactttctatttttaatttatatatttatattaaaaaatttaaattataattatttttatagcacgtgatgaaaaggacccaggtggcacttttcggggaaatgtgcgcggaacccctatttgtttatttttctaaatacattcaaatatgtatccgctcatgagacaataaccctgataaatgcttcaataatattgaaaaaggaagagtatgagtattcaacatttccgtgtcgcccttattcccttttttgcggcattttgccttcctgtttttgctcacccagaaacgctggtgaaagtaaaagatgctgaagatcagttgggtgcacgagtgggttacatcgaactggatctcaacagcggtaagatccttgagagttttcgccccgaagaacgttttccaatgatgagcacttttaaagttctgctatgtggcgcggtattatcccgtgttgacgccgggcaagagcaactcggtcgccgcatacactattctcagaatgacttggttgagtactcaccagtcacagaaaagcatcttacggatggcatgacagtaagagaattatgcagtgctgccataaccatgagtgataacactgcggccaacttacttctgacaacgatcggaggaccgaaggagctaaccgcttttttgcacaacatgggggatcatgtaactcgccttgatcgttgggaaccggagctgaatgaagccataccaaacgacgagcgtgacaccacgatgcctgtagcaatggcaacaacgttgcgcaaactattaactggcgaactacttactctagcttcccggcaacaattaatagactggatggaggcggataaagttgcaggaccacttctgcgctcggcccttccggctggctggtttattgctgataaatctggagccggtgagcgtgggtctcgcggtatcattgcagcactggggccagatggtaagccctcccgtatcgtagttatctacacgacgggcagtcaggcaactatggatgaacgaaatagacagatcgctgagataggtgcctcactgattaagcattggtaactgtcagaccaagtttactcatatatactttagattgatttaaaacttcatttttaatttaaaaggatctaggtgaagatcctttttgataatctcatgaccaaaatcccttaacgtgagttttcgttccactgagcgtcagaccccgtagaaaagatcaaaggatcttcttgagatcctttttttctgcgcgtaatctgctgcttgcaaacaaaaaaaccaccgctaccagcggtggtttgtttgccggatcaagagctaccaactctttttccgaaggtaactggcttcagcagagcgcagataccaaatactgtccttctagtgtagccgtagttaggccaccacttcaagaactctgtagcaccgcctacatacctcgctctgctaatcctgttaccagtggctgctgccagtggcgataagtcgtgtcttaccgggttggactcaagacgatagttaccggataaggcgcagcggtcgggctgaacggggggttcgtgcacacagcccagcttggagcgaacgacctacaccgaactgagatacctacagcgtgagcattgagaaagcgccacgcttcccgaagggagaaaggcggacaggtatccggtaagcggcagggtcggaacaggagagcgcacgagggagcttccaggggggaacgcctggtatctttatagtcctgtcgggtttcgccacctctgacttgagcgtcgatttttgtgatgctcgtcaggggggccgagcctatggaaaaacgccagcaacgcggcctttttacggttcctggccttttgctggccttttgctcacatgttctttcctgcgttatcccctgattctgtggataaccgtattaccgcctttgagtgagctgataccgctcgccgcagccgaacgaccgagcgcagcgagtcagtgagcgaggaagcggaagagcgcccaatacgcaaaccgcctctccccgcgcgttggccgattcattaatgcagctggcacgacaggtttcccgactggaaagcgggcagtgagcgcaacgcaattaatgtgagttacctcactcattaggcaccccaggctttacactttatgcttccggctcctatgttgtgtggaattgtgagcggataacaatttcacacaggaaacagctatgaccatgattacgccaagctcggaattaaccctcactaaagggaacaaaagctggctagt

SEQ ID NO: 82 - protein, 214 aa, artificial
  4D5lp
DIQMTQSPSSLSASVGDRVTITCRASQDVNTAVAWYQQKPGKAPKLLIYSASFLYSGVPSRFSGSRSGTDFTLTISSLQPEDFATYYCQQHYTTPPTFGQGTKVEIKRTVAAPSVFIFPPSDEQLKSGTASVVCLLNNFYPREAKVQWKVDNALQSGNSQESVTEQDSKDSTYSLSSTLTLSKADYEKHKVYACEVTHQGLSSPVTKSFNRGEC